European Patent Specification EP 4 482 578 B1, published December 24, 2025. Title: CRF2 RECEPTOR AGONISTS AND THEIR USE IN THERAPY. Applicant: Corteria Pharmaceuticals. Application WO. The sequence listing filed with the application follows.

SEQUENCE LISTING (244 sequences)

SEQ ID NO: 1 - protein, 38 aa, synthetic construct
  SOURCE 1..38
  VARIANT 1: NOTE = absent or I
  VARIANT 2: NOTE = Valine or D-valine
  VARIANT 7: NOTE = Valine or D-valine
  VARIANT 11: NOTE = L or I or alpha-methyl-leucien or Aib
  MOD_RES 12: NOTE = the epsilon-amino group of the lysine side chain is covalentlybound to an albumin -binding moiety
  VARIANT 13: NOTE = K or Q
  VARIANT 14: NOTE = I or Aib
  VARIANT 15: NOTE = L or alpha-methyl-leucine or Aib
  VARIANT 17: NOTE = E or K
  VARIANT 20: NOTE = K or R
  VARIANT 23: NOTE = K or A or Aib
  VARIANT 25: NOTE = R or alpha-methyl-leucine or Aib
  VARIANT 26: NOTE = E or Aib
  VARIANT 30: NOTE = K or T
  VARIANT 31: NOTE = N or Q or A
  VARIANT 32: NOTE = K or V or T or Aib or E or A or Abu or Nva oralpha-methyl-leucine or Dap or 4-Pip or Thp or Chx or Cpex or Cpx
  VARIANT 36: NOTE = A or E
XXLSLDXPIKXKXXXLXQEXQKXQXXQAEXXXQILXQV

SEQ ID NO: 2 - protein, 38 aa, synthetic construct
  SOURCE 1..38
  MOD_RES 1: NOTE = ACETYLATION
  VARIANT 7: NOTE = D-valine
  MOD_RES 12: NOTE = the epsilon-amino group of the lysine side chain is covalentlybound to an albumin -binding moiety
  MOD_RES 38: NOTE = AMIDATION
IVLSLDXPIKLKQILLKQERQKKQREQAEKNKQILEQV

SEQ ID NO: 3 - protein, 37 aa, synthetic construct
  SOURCE 1..37
  MOD_RES 1: NOTE = ACETYLATION
  VARIANT 6: NOTE = D-valine
  MOD_RES 11: NOTE = the epsilon-amino group of the lysine side chain is covalentlybound to an albumin -binding moiety
  MOD_RES 37: NOTE = AMIDATION
VLSLDXPIKLKQILLKQERQKKQREQAEKNKQILEQV

SEQ ID NO: 4 - protein, 37 aa, synthetic construct; identical to SEQ ID NO: 3
  SOURCE 1..37
  VARIANT 6: NOTE = D-valine
  MOD_RES 11: NOTE = the epsilon-amino group of the lysine side chain is covalentlybound to an albumin -binding moiety
  MOD_RES 37: NOTE = AMIDATION

SEQ ID NO: 5 - protein, 38 aa, synthetic construct; identical to SEQ ID NO: 2
  SOURCE 1..38
  MOD_RES 1: NOTE = met
  VARIANT 7: NOTE = D-valine
  MOD_RES 12: NOTE = the epsilon-amino group of the lysine side chain is covalentlybound to an albumin -binding moiety
  MOD_RES 38: NOTE = AMIDATION

SEQ ID NO: 6 - protein, 37 aa, synthetic construct
  SOURCE 1..37
  MOD_RES 1: NOTE = Acetylated with a propanoyl group
  VARIANT 6: NOTE = D-valine
  MOD_RES 11: NOTE = the epsilon-amino group of the lysine side chain is covalentlybound to an albumin -binding moiety
  MOD_RES 37: NOTE = AMIDATION
VLSLDVPIKLKQILLKQERQKKQREQAEKNKQILEQV

SEQ ID NO: 7 - protein, 37 aa, synthetic construct; identical to SEQ ID NO: 6
  SOURCE 1..37
  MOD_RES 1: NOTE = Acetylated with a butanoyl group
  VARIANT 6: NOTE = D-valine
  MOD_RES 11: NOTE = the epsilon-amino group of the lysine side chain is covalentlybound to an albumin -binding moiety
  MOD_RES 37: NOTE = AMIDATION

SEQ ID NO: 8 - protein, 37 aa, synthetic construct; identical to SEQ ID NO: 6
  SOURCE 1..37
  MOD_RES 1: NOTE = Acetylated with a pentanoyl group
  VARIANT 6: NOTE = D-valine
  MOD_RES 11: NOTE = the epsilon-amino group of the lysine side chain is covalentlybound to an albumin -binding moiety
  MOD_RES 37: NOTE = AMIDATION

SEQ ID NO: 9 - protein, 37 aa, synthetic construct; identical to SEQ ID NO: 6
  SOURCE 1..37
  MOD_RES 1: NOTE = Acetylated with a isopentanoyl group
  VARIANT 6: NOTE = D-valine
  MOD_RES 11: NOTE = the epsilon-amino group of the lysine side chain is covalentlybound to an albumin -binding moiety
  MOD_RES 37: NOTE = AMIDATION

SEQ ID NO: 10 - protein, 38 aa, synthetic construct
  SOURCE 1..38
  VARIANT 7: NOTE = D-valine
  MOD_RES 12: NOTE = the epsilon-amino group of the lysine side chain is covalentlybound to an albumin -binding moiety
  VARIANT 32: NOTE = X is Aib
  MOD_RES 38: NOTE = AMIDATION
IVLSLDVPIKLKQILLKQERQKKQREQAEKNXQILEQV

SEQ ID NO: 11 - protein, 38 aa, synthetic construct
  SOURCE 1..38
  VARIANT 7: NOTE = D-valine
  MOD_RES 12: NOTE = the epsilon-amino group of the lysine side chain is covalentlybound to an albumin -binding moiety
  VARIANT 32: NOTE = X is Aib
  MOD_RES 38: NOTE = AMIDATION
IVLSLDVPIKLKKILLEQEKQKKQREQAETNXQILAQV

SEQ ID NO: 12 - protein, 38 aa, synthetic construct; identical to SEQ ID NO: 11
  SOURCE 1..38
  VARIANT 7: NOTE = D-valine
  MOD_RES 12: NOTE = the epsilon-amino group of the lysine side chain is covalentlybound to an albumin -binding moiety
  VARIANT 32: NOTE = X is Aib
  MOD_RES 38: NOTE = AMIDATION

SEQ ID NO: 13 - protein, 38 aa, synthetic construct
  SOURCE 1..38
  VARIANT 7: NOTE = D-valine
  MOD_RES 12: NOTE = the epsilon-amino group of the lysine side chain is covalentlybound to an albumin -binding moiety
  MOD_RES 38: NOTE = AMIDATION
IVLSLDVPIKLKQILLKQERQKKQREQAEKNVQILEQV

SEQ ID NO: 14 - protein, 38 aa, synthetic construct
  SOURCE 1..38
  VARIANT 7: NOTE = D-valine
  MOD_RES 12: NOTE = the epsilon-amino group of the lysine side chain is covalentlybound to an albumin -binding moiety
  MOD_RES 38: NOTE = AMIDATION
IVLSLDVPIKLKQILLKQERQKKQREQAEKNTQILEQV

SEQ ID NO: 15 - protein, 37 aa, synthetic construct
  SOURCE 1..37
  VARIANT 6: NOTE = D-valine
  MOD_RES 11: NOTE = the epsilon-amino group of the lysine side chain is covalentlybound to an albumin -binding moiety
  VARIANT 22: NOTE = X is Aib
  VARIANT 31: NOTE = X is Aib
  MOD_RES 37: NOTE = AMIDATION
VLSLDVPIKLKKILLEQEKQKXQREQAETNXQILAQV

SEQ ID NO: 16 - protein, 38 aa, synthetic construct; identical to SEQ ID NO: 10
  SOURCE 1..38
  MOD_RES 1: NOTE = ACETYLATION
  VARIANT 7: NOTE = D-valine
  MOD_RES 12: NOTE = the epsilon-amino group of the lysine side chain is covalentlybound to an albumin -binding moiety
  VARIANT 32: NOTE = X is Aib
  MOD_RES 38: NOTE = AMIDATION

SEQ ID NO: 17 - protein, 38 aa, synthetic construct
  SOURCE 1..38
  MOD_RES 1: NOTE = ACETYLATION
  VARIANT 7: NOTE = D-valine
  MOD_RES 12: NOTE = the epsilon-amino group of the lysine side chain is covalentlybound to an albumin -binding moiety
  MOD_RES 38: NOTE = AMIDATION
IVLSLDVPIKLKQILLKQERQKKQREQAEKNEQILEQV

SEQ ID NO: 18 - protein, 38 aa, synthetic construct
  SOURCE 1..38
  MOD_RES 1: NOTE = ACETYLATION
  VARIANT 7: NOTE = D-valine
  MOD_RES 12: NOTE = the epsilon-amino group of the lysine side chain is covalentlybound to an albumin -binding moiety
  VARIANT 14: NOTE = X is Aib
  MOD_RES 38: NOTE = AMIDATION
IVLSLDVPIKLKQXLLKQERQKKQREQAEKNVQILEQV

SEQ ID NO: 19 - protein, 38 aa, synthetic construct
  SOURCE 1..38
  MOD_RES 1: NOTE = ACETYLATION
  VARIANT 11: NOTE = X is alpha-methyl-leucine
  MOD_RES 12: NOTE = the epsilon-amino group of the lysine side chain is covalentlybound to an albumin -binding moiety
  VARIANT 32: NOTE = X is Aib
  MOD_RES 38: NOTE = AMIDATION
IVLSLDVPIKXKQILLKQERQKKQREQAEKNXQILEQV

SEQ ID NO: 20 - protein, 38 aa, synthetic construct
  SOURCE 1..38
  MOD_RES 1: NOTE = ACETYLATION
  VARIANT 11: NOTE = X is alpha-methyl-leucine
  MOD_RES 12: NOTE = the epsilon-amino group of the lysine side chain is covalentlybound to an albumin -binding moiety
  VARIANT 14: NOTE = X is Aib
  VARIANT 32: NOTE = X is Aib
  MOD_RES 38: NOTE = AMIDATION
IVLSLDVPIKXKQXLLKQERQKKQREQAEKNXQILEQV

SEQ ID NO: 21 - protein, 38 aa, synthetic construct
  SOURCE 1..38
  MOD_RES 1: NOTE = ACETYLATION
  VARIANT 7: NOTE = D-valine
  MOD_RES 12: NOTE = the epsilon-amino group of the lysine side chain is covalentlybound to an albumin -binding moiety
  VARIANT 32: NOTE = X is Aib
  MOD_RES 38: NOTE = AMIDATION
IVLSLDVPIKLKKILLKQERQKKQREQAEKNXQILEQV

SEQ ID NO: 22 - protein, 37 aa, synthetic construct
  SOURCE 1..37
  MOD_RES 1: NOTE = Acetylated with a pentanoyl group
  VARIANT 6: NOTE = D-valine
  MOD_RES 11: NOTE = the epsilon-amino group of the lysine side chain is covalentlybound to an albumin -binding moiety
  VARIANT 13: NOTE = X is Aib
  MOD_RES 37: NOTE = AMIDATION
VLSLDVPIKLKQXLLKQERQKKQREQAEKNVQILEQV

SEQ ID NO: 23 - protein, 38 aa, synthetic construct; identical to SEQ ID NO: 10
  SOURCE 1..38
  MOD_RES 1: NOTE = METHYLATION
  VARIANT 7: NOTE = D-valine
  MOD_RES 12: NOTE = the epsilon-amino group of the lysine side chain is covalentlybound to an albumin -binding moiety
  VARIANT 32: NOTE = X is Aib
  MOD_RES 38: NOTE = AMIDATION

SEQ ID NO: 24 - protein, 38 aa, synthetic construct
  SOURCE 1..38
  MOD_RES 1: NOTE = METHYLATION
  VARIANT 7: NOTE = D-valine
  MOD_RES 12: NOTE = the epsilon-amino group of the lysine side chain is covalentlybound to an albumin -binding moiety
  MOD_RES 38: NOTE = AMIDATION
IVLSLDVPIKLKQILLKQERQKKQREQAEKNAQILEQV

SEQ ID NO: 25 - protein, 38 aa, synthetic construct
  SOURCE 1..38
  MOD_RES 12: NOTE = the epsilon-amino group of the lysine side chain is covalentlybound to an albumin -binding moiety
  VARIANT 14: NOTE = X is Aib
  VARIANT 32: NOTE = X is Aib
  MOD_RES 38: NOTE = AMIDATION
IVLSLDVPIKLKQXLLKQERQKKQREQAEKNXQILEQV

SEQ ID NO: 26 - protein, 38 aa, synthetic construct; identical to SEQ ID NO: 25
  SOURCE 1..38
  MOD_RES 1: NOTE = ACETYLATION
  MOD_RES 12: NOTE = the epsilon-amino group of the lysine side chain is covalentlybound to an albumin -binding moiety
  VARIANT 14: NOTE = X is Aib
  VARIANT 32: NOTE = X is Aib
  MOD_RES 38: NOTE = AMIDATION

SEQ ID NO: 27 - protein, 38 aa, synthetic construct; identical to SEQ ID NO: 18
  SOURCE 1..38
  MOD_RES 1: NOTE = ACETYLATION
  VARIANT 7: NOTE = D-valine
  MOD_RES 12: NOTE = the epsilon-amino group of the lysine side chain is covalentlybound to an albumin -binding moiety
  VARIANT 14: NOTE = X is Aib
  MOD_RES 38: NOTE = AMIDATION

SEQ ID NO: 28 - protein, 38 aa, synthetic construct; identical to SEQ ID NO: 18
  SOURCE 1..38
  MOD_RES 1: NOTE = METHYLATION
  VARIANT 7: NOTE = D-valine
  MOD_RES 12: NOTE = the epsilon-amino group of the lysine side chain is covalentlybound to an albumin -binding moiety
  VARIANT 14: NOTE = X is Aib
  MOD_RES 38: NOTE = AMIDATION

SEQ ID NO: 29 - protein, 37 aa, synthetic construct; identical to SEQ ID NO: 22
  SOURCE 1..37
  MOD_RES 1: NOTE = Acetylated with a pentanoyl group
  VARIANT 6: NOTE = D-valine
  MOD_RES 11: NOTE = the epsilon-amino group of the lysine side chain is covalentlybound to an albumin -binding moiety
  VARIANT 13: NOTE = X is Aib
  MOD_RES 37: NOTE = AMIDATION

SEQ ID NO: 30 - protein, 38 aa, synthetic construct; identical to SEQ ID NO: 10
  SOURCE 1..38
  MOD_RES 1: NOTE = ACETYLATION
  VARIANT 7: NOTE = D-valine
  MOD_RES 12: NOTE = the epsilon-amino group of the lysine side chain is covalentlybound to an albumin -binding moiety
  VARIANT 32: NOTE = X is Aib
  MOD_RES 38: NOTE = AMIDATION

SEQ ID NO: 31 - protein, 38 aa, synthetic construct; identical to SEQ ID NO: 10
  SOURCE 1..38
  MOD_RES 1: NOTE = METHYLATION
  VARIANT 7: NOTE = D-valine
  MOD_RES 12: NOTE = the epsilon-amino group of the lysine side chain is covalentlybound to an albumin -binding moiety
  VARIANT 32: NOTE = X is Aib
  MOD_RES 38: NOTE = AMIDATION

SEQ ID NO: 32 - protein, 37 aa, synthetic construct
  SOURCE 1..37
  MOD_RES 1: NOTE = Acetylated with a pentanoyl group
  VARIANT 6: NOTE = D-valine
  MOD_RES 11: NOTE = the epsilon-amino group of the lysine side chain is covalentlybound to an albumin -binding moiety
  VARIANT 31: NOTE = X is Aib
  MOD_RES 37: NOTE = AMIDATION
VLSLDVPIKLKQILLKQERQKKQREQAEKNXQILEQV

SEQ ID NO: 33 - protein, 37 aa, synthetic construct
  SOURCE 1..37
  MOD_RES 1: NOTE = ACETYLATION
  VARIANT 6: NOTE = D-valine
  MOD_RES 11: NOTE = the epsilon-amino group of the lysine side chain is covalentlybound to an albumin -binding moiety
  MOD_RES 37: NOTE = AMIDATION
VLSLDVPIKLKKILLEQEKQKKQREQAETNKQILAQV

SEQ ID NO: 34 - protein, 37 aa, synthetic construct; identical to SEQ ID NO: 33
  SOURCE 1..37
  VARIANT 6: NOTE = D-valine
  VARIANT 11: NOTE = the epsilon-amino group of the lysine side chain is covalentlybound to an albumin -binding moiety
  MOD_RES 37: NOTE = AMIDATION

SEQ ID NO: 35 - protein, 37 aa, synthetic construct; identical to SEQ ID NO: 33
  SOURCE 1..37
  MOD_RES 1: NOTE = Acetylated with a propanoyl group
  VARIANT 6: NOTE = D-valine
  MOD_RES 11: NOTE = the epsilon-amino group of the lysine side chain is covalentlybound to an albumin -binding moiety
  MOD_RES 37: NOTE = AMIDATION

SEQ ID NO: 36 - protein, 37 aa, synthetic construct; identical to SEQ ID NO: 33
  SOURCE 1..37
  MOD_RES 1: NOTE = Acetylated with a butanoyl group
  VARIANT 6: NOTE = D-valine
  MOD_RES 11: NOTE = the epsilon-amino group of the lysine side chain is covalentlybound to an albumin -binding moiety
  MOD_RES 37: NOTE = AMIDATION

SEQ ID NO: 37 - protein, 37 aa, synthetic construct; identical to SEQ ID NO: 33
  SOURCE 1..37
  MOD_RES 1: NOTE = Acetylated with a pentanoyl group
  VARIANT 6: NOTE = D-valine
  MOD_RES 11: NOTE = the epsilon-amino group of the lysine side chain is covalentlybound to an albumin -binding moiety
  MOD_RES 37: NOTE = AMIDATION

SEQ ID NO: 38 - protein, 38 aa, synthetic construct
  SOURCE 1..38
  VARIANT 11: NOTE = X is alpha-methyl-leucine
  MOD_RES 12: NOTE = the epsilon-amino group of the lysine side chain is covalentlybound to an albumin -binding moiety
  VARIANT 32: NOTE = X is Aib
  MOD_RES 38: NOTE = AMIDATION
IVLSLDVPIKXKKILLEQEKQKKQREQAETNXQILAQV

SEQ ID NO: 39 - protein, 38 aa, synthetic construct; identical to SEQ ID NO: 11
  SOURCE 1..38
  MOD_RES 1: NOTE = ACETYLATION
  MOD_RES 12: NOTE = the epsilon-amino group of the lysine side chain is covalentlybound to an albumin -binding moiety
  VARIANT 32: NOTE = X is Aib
  MOD_RES 38: NOTE = AMIDATION

SEQ ID NO: 40 - protein, 38 aa, synthetic construct; identical to SEQ ID NO: 11
  SOURCE 1..38
  MOD_RES 1: NOTE = ACETYLATION
  VARIANT 7: NOTE = D-valine
  MOD_RES 12: NOTE = the epsilon-amino group of the lysine side chain is covalentlybound to an albumin -binding moiety
  VARIANT 32: NOTE = X is Aib
  MOD_RES 38: NOTE = AMIDATION

SEQ ID NO: 41 - protein, 38 aa, synthetic construct; identical to SEQ ID NO: 11
  SOURCE 1..38
  MOD_RES 1: NOTE = ACETYLATION
  VARIANT 7: NOTE = D-valine
  MOD_RES 12: NOTE = the epsilon-amino group of the lysine side chain is covalentlybound to an albumin -binding moiety
  VARIANT 32: NOTE = x is Aib
  MOD_RES 38: NOTE = AMIDATION

SEQ ID NO: 42 - protein, 38 aa, synthetic construct; identical to SEQ ID NO: 11
  SOURCE 1..38
  MOD_RES 1: NOTE = ACETYLATION
  VARIANT 7: NOTE = D-valine
  MOD_RES 12: NOTE = the epsilon-amino group of the lysine side chain is covalentlybound to an albumin -binding moiety
  VARIANT 32: NOTE = X is Aib
  MOD_RES 38: NOTE = AMIDATION

SEQ ID NO: 43 - protein, 38 aa, synthetic construct; identical to SEQ ID NO: 38
  SOURCE 1..38
  MOD_RES 1: NOTE = ACETYLATION
  VARIANT 11: NOTE = X is alpha-methyl-leucine
  MOD_RES 12: NOTE = the epsilon-amino group of the lysine side chain is covalentlybound to an albumin -binding moiety
  VARIANT 32: NOTE = X is Aib
  MOD_RES 38: NOTE = AMIDATION

SEQ ID NO: 44 - protein, 38 aa, synthetic construct; identical to SEQ ID NO: 38
  SOURCE 1..38
  MOD_RES 1: NOTE = ACETYLATION
  VARIANT 7: NOTE = D-valine
  VARIANT 11: NOTE = X is alpha-methyl-leucine
  MOD_RES 12: NOTE = the epsilon-amino group of the lysine side chain is covalentlybound to an albumin -binding moiety
  VARIANT 32: NOTE = X is Aib
  MOD_RES 38: NOTE = AMIDATION

SEQ ID NO: 45 - protein, 37 aa, synthetic construct
  SOURCE 1..37
  MOD_RES 1: NOTE = ACETYLATION
  VARIANT 6: NOTE = D-valine
  MOD_RES 11: NOTE = the epsilon-amino group of the lysine side chain is covalentlybound to an albumin -binding moiety
  VARIANT 31: NOTE = X is Aib
  MOD_RES 37: NOTE = AMIDATION
VLSLDVPIKLKKILLEQEKQKKQREQAETNXQILAQV

SEQ ID NO: 46 - protein, 37 aa, synthetic construct
  SOURCE 1..37
  MOD_RES 1: NOTE = ACETYLATION
  VARIANT 6: NOTE = D-valine
  VARIANT 10: NOTE = X is alpha-methyl-leucine
  MOD_RES 11: NOTE = the epsilon-amino group of the lysine side chain is covalentlybound to an albumin -binding moiety
  VARIANT 31: NOTE = X is Aib
  MOD_RES 37: NOTE = AMIDATION
VLSLDVPIKXKKILLEQEKQKKQREQAETNXQILAQV

SEQ ID NO: 47 - protein, 38 aa, synthetic construct
  SOURCE 1..38
  MOD_RES 1: NOTE = ACETYLATION
  VARIANT 7: NOTE = D-valine
  MOD_RES 12: NOTE = the epsilon-amino group of the lysine side chain is covalentlybound to an albumin -binding moiety
  MOD_RES 38: NOTE = AMIDATION
IVLSLDVPIKLKKILLEQEKQKKQREQAETNAQILAQV

SEQ ID NO: 48 - protein, 38 aa, synthetic construct
  SOURCE 1..38
  MOD_RES 1: NOTE = ACETYLATION
  VARIANT 7: NOTE = D-valine
  MOD_RES 12: NOTE = the epsilon-amino group of the lysine side chain is covalentlybound to an albumin -binding moiety
  MOD_RES 38: NOTE = AMIDATION
IVLSLDVPIKLKKILLEQEKQKKQREQAETNVQILAQV

SEQ ID NO: 49 - protein, 38 aa, synthetic construct
  SOURCE 1..38
  MOD_RES 1: NOTE = ACETYLATION
  VARIANT 11: NOTE = X is alpha-methyl-leucine
  MOD_RES 12: NOTE = the epsilon-amino group of the lysine side chain is covalentlybound to an albumin -binding moiety
  MOD_RES 38: NOTE = ACETYLATION
IVLSLDVPIKXKKILLEQEKQKKQREQAETNVQILAQV

SEQ ID NO: 50 - protein, 38 aa, synthetic construct; identical to SEQ ID NO: 49
  SOURCE 1..38
  MOD_RES 1: NOTE = ACETYLATION
  VARIANT 7: NOTE = D-valine
  VARIANT 11: NOTE = X is alpha-methyl-leucine
  MOD_RES 12: NOTE = the epsilon-amino group of the lysine side chain is covalentlybound to an albumin -binding moiety
  MOD_RES 38: NOTE = AMIDATION

SEQ ID NO: 51 - protein, 38 aa, synthetic construct; identical to SEQ ID NO: 11
  SOURCE 1..38
  MOD_RES 1: NOTE = ACETYLATION
  VARIANT 7: NOTE = D-valine
  MOD_RES 12: NOTE = the epsilon-amino group of the lysine side chain is covalentlybound to an albumin -binding moiety
  VARIANT 32: NOTE = X is Abu
  MOD_RES 38: NOTE = AMIDATION

SEQ ID NO: 52 - protein, 38 aa, synthetic construct; identical to SEQ ID NO: 11
  SOURCE 1..38
  MOD_RES 1: NOTE = ACETYLATION
  VARIANT 7: NOTE = D-valine
  MOD_RES 12: NOTE = the epsilon-amino group of the lysine side chain is covalentlybound to an albumin -binding moiety
  VARIANT 32: NOTE = X is Nva
  MOD_RES 38: NOTE = AMIDATION

SEQ ID NO: 53 - protein, 38 aa, synthetic construct
  SOURCE 1..38
  MOD_RES 1: NOTE = ACETYLATION
  VARIANT 7: NOTE = D-valine
  VARIANT 11: NOTE = X is alpha-methyl-leucine
  MOD_RES 12: NOTE = the epsilon-amino group of the lysine side chain is covalentlybound to an albumin -binding moiety
  MOD_RES 38: NOTE = AMIDATION
IVLSLDVPIKXKKILLEQEKQKKQREQAETDKQILAQV

SEQ ID NO: 54 - protein, 39 aa, synthetic construct
  SOURCE 1..39
  MOD_RES 1: NOTE = ACETYLATION
  VARIANT 7: NOTE = D-valine
  MOD_RES 12: NOTE = the epsilon-amino group of the lysine side chain is covalentlybound to an albumin -binding moiety
  VARIANT 32: NOTE = X is alpha-methyl-leucine
  MOD_RES 38: NOTE = AMIDATION
IVLSLDVPIKLKKILLEQEKQKKQREQAETNXKQILAQV

SEQ ID NO: 55 - protein, 38 aa, synthetic construct; identical to SEQ ID NO: 11
  SOURCE 1..38
  MOD_RES 1: NOTE = ACETYLATION
  VARIANT 7: NOTE = D-valine
  MOD_RES 12: NOTE = the epsilon-amino group of the lysine side chain is covalentlybound to an albumin -binding moiety
  VARIANT 32: NOTE = X is Dap
  MOD_RES 38: NOTE = AMIDATION

SEQ ID NO: 56 - protein, 38 aa, synthetic construct
  SOURCE 1..38
  MOD_RES 1: NOTE = ACETYLATION
  VARIANT 7: NOTE = D-valine
  MOD_RES 12: NOTE = the epsilon-amino group of the lysine side chain is covalentlybound to an albumin -binding moiety
  MOD_RES 38: NOTE = AMIDATION
IVLSLDVPIKLKKILLEQEKQKKQREQAETNEQILAQV

SEQ ID NO: 57 - protein, 38 aa, synthetic construct; identical to SEQ ID NO: 11
  SOURCE 1..38
  MOD_RES 1: NOTE = ACETYLATION
  VARIANT 7: NOTE = D-valine
  MOD_RES 12: NOTE = the epsilon-amino group of the lysine side chain is covalentlybound to an albumin -binding moiety
  VARIANT 32: NOTE = X is 4-Pip
  MOD_RES 38: NOTE = AMIDATION

SEQ ID NO: 58 - protein, 38 aa, synthetic construct; identical to SEQ ID NO: 11
  SOURCE 1..38
  MOD_RES 1: NOTE = ACETYLATION
  VARIANT 7: NOTE = D-valine
  MOD_RES 12: NOTE = the epsilon-amino group of the lysine side chain is covalentlybound to an albumin -binding moiety
  VARIANT 32: NOTE = X is Thp
  MOD_RES 38: NOTE = AMIDATION

SEQ ID NO: 59 - protein, 38 aa, synthetic construct; identical to SEQ ID NO: 11
  SOURCE 1..38
  MOD_RES 1: NOTE = ACETYLATION
  VARIANT 7: NOTE = D-valine
  MOD_RES 12: NOTE = the epsilon-amino group of the lysine side chain is covalentlybound to an albumin -binding moiety
  VARIANT 32: NOTE = X is Chx
  MOD_RES 38: NOTE = AMIDATION

SEQ ID NO: 60 - protein, 38 aa, synthetic construct; identical to SEQ ID NO: 11
  SOURCE 1..38
  MOD_RES 1: NOTE = ACETYLATION
  VARIANT 7: NOTE = D-valine
  MOD_RES 12: NOTE = the epsilon-amino group of the lysine side chain is covalentlybound to an albumin -binding moiety
  VARIANT 32: NOTE = X is Cpex
  MOD_RES 38: NOTE = AMIDATION

SEQ ID NO: 61 - protein, 38 aa, synthetic construct; identical to SEQ ID NO: 11
  SOURCE 1..38
  MOD_RES 1: NOTE = ACETYLATION
  VARIANT 7: NOTE = D-valine
  MOD_RES 12: NOTE = the epsilon-amino group of the lysine side chain is covalentlybound to an albumin -binding moiety
  VARIANT 32: NOTE = X is Cpx
  MOD_RES 38: NOTE = AMIDATION

SEQ ID NO: 62 - protein, 38 aa, synthetic construct
  SOURCE 1..38
  MOD_RES 1: NOTE = ACETYLATION
  VARIANT 7: NOTE = D-valine
  MOD_RES 12: NOTE = the epsilon-amino group of the lysine side chain is covalentlybound to an albumin -binding moiety
  VARIANT 32: NOTE = X is 4-Pip
  MOD_RES 38: NOTE = AMIDATION
IVLSLDVPIKLKKILLEQEKQKAQREQAETNXQILAQV

SEQ ID NO: 63 - protein, 38 aa, synthetic construct
  SOURCE 1..38
  MOD_RES 1: NOTE = ACETYLATION
  VARIANT 7: NOTE = D-valine
  MOD_RES 12: NOTE = the epsilon-amino group of the lysine side chain is covalentlybound to an albumin -binding moiety
  VARIANT 23: NOTE = X is Aib
  VARIANT 32: NOTE = X is 4-Pip
IVLSLDVPIKLKKILLEQEKQKXQREQAETNXQILAQV

SEQ ID NO: 64 - protein, 38 aa, synthetic construct; identical to SEQ ID NO: 11
  SOURCE 1..38
  MOD_RES 1: NOTE = METHYLATION
  VARIANT 7: NOTE = D-valine
  MOD_RES 12: NOTE = the epsilon-amino group of the lysine side chain is covalentlybound to an albumin -binding moiety
  VARIANT 32: NOTE = X is Aib
  MOD_RES 38: NOTE = AMIDATION

SEQ ID NO: 65 - protein, 38 aa, synthetic construct; identical to SEQ ID NO: 38
  SOURCE 1..38
  MOD_RES 1: NOTE = METHYLATION
  VARIANT 7: NOTE = D-valine
  VARIANT 11: NOTE = X is alpha-methyl-leucine
  MOD_RES 12: NOTE = the epsilon-amino group of the lysine side chain is covalentlybound to an albumin -binding moiety
  VARIANT 32: NOTE = X is Aib
  MOD_RES 38: NOTE = AMIDATION

SEQ ID NO: 66 - protein, 38 aa, synthetic construct; identical to SEQ ID NO: 48
  SOURCE 1..38
  MOD_RES 1: NOTE = METHYLATION
  VARIANT 7: NOTE = D-valine
  MOD_RES 12: NOTE = the epsilon-amino group of the lysine side chain is covalentlybound to an albumin -binding moiety
  MOD_RES 38: NOTE = AMIDATION

SEQ ID NO: 67 - protein, 38 aa, synthetic construct; identical to SEQ ID NO: 49
  SOURCE 1..38
  MOD_RES 1: NOTE = METHYLATION
  VARIANT 7: NOTE = D-valine
  VARIANT 11: NOTE = X is alpha-methyl-leucine
  MOD_RES 12: NOTE = the epsilon-amino group of the lysine side chain is covalentlybound to an albumin -binding moiety
  MOD_RES 38: NOTE = AMIDATION

SEQ ID NO: 68 - protein, 38 aa, synthetic construct; identical to SEQ ID NO: 47
  SOURCE 1..38
  MOD_RES 1: NOTE = METHYLATION
  VARIANT 7: NOTE = D-valine
  MOD_RES 12: NOTE = the epsilon-amino group of the lysine side chain is covalentlybound to an albumin -binding moiety
  MOD_RES 38: NOTE = AMIDATION

SEQ ID NO: 69 - protein, 38 aa, synthetic construct; identical to SEQ ID NO: 11
  SOURCE 1..38
  MOD_RES 1: NOTE = METHYLATION
  VARIANT 7: NOTE = D-valine
  MOD_RES 12: NOTE = the epsilon-amino group of the lysine side chain is covalentlybound to an albumin -binding moiety
  VARIANT 32: NOTE = X is Abu
  MOD_RES 38: NOTE = AMIDATION

SEQ ID NO: 70 - protein, 38 aa, synthetic construct; identical to SEQ ID NO: 11
  SOURCE 1..38
  MOD_RES 1: NOTE = METHYLATION
  VARIANT 7: NOTE = D-valine
  MOD_RES 12: NOTE = the epsilon-amino group of the lysine side chain is covalentlybound to an albumin -binding moiety
  VARIANT 32: NOTE = X is Dap
  MOD_RES 38: NOTE = AMIDATION

SEQ ID NO: 71 - protein, 38 aa, synthetic construct; identical to SEQ ID NO: 56
  SOURCE 1..38
  MOD_RES 1: NOTE = METHYLATION
  VARIANT 7: NOTE = D-valine
  MOD_RES 12: NOTE = the epsilon-amino group of the lysine side chain is covalentlybound to an albumin -binding moiety
  MOD_RES 38: NOTE = AMIDATION

SEQ ID NO: 72 - protein, 38 aa, synthetic construct; identical to SEQ ID NO: 11
  SOURCE 1..38
  MOD_RES 1: NOTE = METHYLATION
  VARIANT 7: NOTE = D-valine
  MOD_RES 12: NOTE = the epsilon-amino group of the lysine side chain is covalentlybound to an albumin -binding moiety
  VARIANT 32: NOTE = X is 4-Pip
  MOD_RES 38: NOTE = AMIDATION

SEQ ID NO: 73 - protein, 38 aa, synthetic construct; identical to SEQ ID NO: 11
  SOURCE 1..38
  MOD_RES 1: NOTE = METHYLATION
  VARIANT 7: NOTE = D-valine
  MOD_RES 12: NOTE = the epsilon-amino group of the lysine side chain is covalentlybound to an albumin -binding moiety
  VARIANT 32: NOTE = X is Thp
  MOD_RES 38: NOTE = AMIDATION

SEQ ID NO: 74 - protein, 38 aa, synthetic construct; identical to SEQ ID NO: 62
  SOURCE 1..38
  MOD_RES 1: NOTE = METHYLATION
  VARIANT 7: NOTE = D-valine
  MOD_RES 12: NOTE = the epsilon-amino group of the lysine side chain is covalentlybound to an albumin -binding moiety
  VARIANT 32: NOTE = X is Aib
  MOD_RES 38: NOTE = AMIDATION

SEQ ID NO: 75 - protein, 38 aa, synthetic construct; identical to SEQ ID NO: 63
  SOURCE 1..38
  MOD_RES 1: NOTE = METHYLATION
  VARIANT 7: NOTE = D-valine
  MOD_RES 12: NOTE = the epsilon-amino group of the lysine side chain is covalentlybound to an albumin -binding moiety
  VARIANT 23: NOTE = X is Aib
  VARIANT 32: NOTE = X is Aib

SEQ ID NO: 76 - protein, 38 aa, synthetic construct; identical to SEQ ID NO: 62
  SOURCE 1..38
  MOD_RES 1: NOTE = METHYLATION
  VARIANT 7: NOTE = D-valine
  MOD_RES 12: NOTE = the epsilon-amino group of the lysine side chain is covalentlybound to an albumin -binding moiety
  VARIANT 32: NOTE = X is 4-Pip
  MOD_RES 38: NOTE = AMIDATION

SEQ ID NO: 77 - protein, 38 aa, synthetic construct; identical to SEQ ID NO: 63
  SOURCE 1..38
  MOD_RES 1: NOTE = METHYLATION
  VARIANT 7: NOTE = D-valine
  MOD_RES 12: NOTE = the epsilon-amino group of the lysine side chain is covalentlybound to an albumin -binding moiety
  VARIANT 23: NOTE = X is Aib
  VARIANT 32: NOTE = X is 4-Pip

SEQ ID NO: 78 - protein, 37 aa, synthetic construct; identical to SEQ ID NO: 45
  SOURCE 1..37
  MOD_RES 1: NOTE = Acetylated with a propanoyl group
  VARIANT 6: NOTE = D-valine
  MOD_RES 11: NOTE = the epsilon-amino group of the lysine side chain is covalentlybound to an albumin -binding moiety
  VARIANT 31: NOTE = X is Aib
  MOD_RES 37: NOTE = AMIDATION

SEQ ID NO: 79 - protein, 37 aa, synthetic construct; identical to SEQ ID NO: 45
  SOURCE 1..37
  MOD_RES 1: NOTE = Acetylated with a butanoyl group
  VARIANT 6: NOTE = D-valine
  MOD_RES 11: NOTE = the epsilon-amino group of the lysine side chain is covalentlybound to an albumin -binding moiety
  VARIANT 31: NOTE = X is Aib
  MOD_RES 37: NOTE = AMIDATION

SEQ ID NO: 80 - protein, 37 aa, synthetic construct; identical to SEQ ID NO: 45
  SOURCE 1..37
  MOD_RES 1: NOTE = Acetylated with a pentanoyl group
  VARIANT 6: NOTE = D-valine
  MOD_RES 11: NOTE = the epsilon-amino group of the lysine side chain is covalentlybound to an albumin -binding moiety
  VARIANT 31: NOTE = X is Aib
  MOD_RES 37: NOTE = AMIDATION

SEQ ID NO: 81 - protein, 37 aa, synthetic construct
  SOURCE 1..37
  MOD_RES 1: NOTE = Acetylated with a pentanoyl group
  VARIANT 6: NOTE = D-valine
  MOD_RES 11: NOTE = the epsilon-amino group of the lysine side chain is covalentlybound to an albumin -binding moiety
  MOD_RES 37: NOTE = AMIDATION
VLSLDVPIKLKKILLEQEKQKKQREQAETNVQILAQV

SEQ ID NO: 82 - protein, 38 aa, synthetic construct; identical to SEQ ID NO: 11
  SOURCE 1..38
  MOD_RES 1: NOTE = ACETYLATION
  VARIANT 7: NOTE = D-valine
  MOD_RES 12: NOTE = the epsilon-amino group of the lysine side chain is covalentlybound to an albumin -binding moiety
  VARIANT 32: NOTE = X is Aib
  MOD_RES 38: NOTE = AMIDATION

SEQ ID NO: 83 - protein, 38 aa, synthetic construct; identical to SEQ ID NO: 11
  SOURCE 1..38
  MOD_RES 1: NOTE = ACETYLATION
  VARIANT 7: NOTE = D-valine
  MOD_RES 12: NOTE = the epsilon-amino group of the lysine side chain is covalentlybound to an albumin -binding moiety
  VARIANT 32: NOTE = X is Abu
  MOD_RES 38: NOTE = AMIDATION

SEQ ID NO: 84 - protein, 38 aa, synthetic construct; identical to SEQ ID NO: 11
  SOURCE 1..38
  MOD_RES 1: NOTE = ACETYLATION
  VARIANT 7: NOTE = D-valine
  MOD_RES 12: NOTE = the epsilon-amino group of the lysine side chain is covalentlybound to an albumin -binding moiety
  VARIANT 32: NOTE = X is 4-Pip
  MOD_RES 38: NOTE = AMIDATION

SEQ ID NO: 85 - protein, 38 aa, synthetic construct; identical to SEQ ID NO: 56
  SOURCE 1..38
  MOD_RES 1: NOTE = ACETYLATION
  VARIANT 7: NOTE = D-valine
  MOD_RES 12: NOTE = the epsilon-amino group of the lysine side chain is covalentlybound to an albumin -binding moiety
  MOD_RES 38: NOTE = AMIDATION

SEQ ID NO: 86 - protein, 37 aa, synthetic construct; identical to SEQ ID NO: 45
  SOURCE 1..37
  MOD_RES 1: NOTE = Acetylated with a pentanoyl group
  VARIANT 6: NOTE = D-valine
  MOD_RES 11: NOTE = the epsilon-amino group of the lysine side chain is covalentlybound to an albumin -binding moiety
  VARIANT 31: NOTE = X is Aib
  MOD_RES 37: NOTE = AMIDATION

SEQ ID NO: 87 - protein, 38 aa, synthetic construct; identical to SEQ ID NO: 11
  SOURCE 1..38
  MOD_RES 1: NOTE = METHYLATION
  VARIANT 7: NOTE = D-valine
  MOD_RES 12: NOTE = the epsilon-amino group of the lysine side chain is covalentlybound to an albumin -binding moiety
  VARIANT 32: NOTE = X is Aib
  MOD_RES 38: NOTE = AMIDATION

SEQ ID NO: 88 - protein, 38 aa, synthetic construct; identical to SEQ ID NO: 62
  SOURCE 1..38
  MOD_RES 1: NOTE = METHYLATION
  VARIANT 7: NOTE = D-valine
  MOD_RES 12: NOTE = the epsilon-amino group of the lysine side chain is covalentlybound to an albumin -binding moiety
  VARIANT 32: NOTE = X is Aib
  MOD_RES 38: NOTE = AMIDATION

SEQ ID NO: 89 - protein, 38 aa, synthetic construct; identical to SEQ ID NO: 63
  SOURCE 1..38
  MOD_RES 1: NOTE = METHYLATION
  VARIANT 7: NOTE = D-valine
  MOD_RES 12: NOTE = the epsilon-amino group of the lysine side chain is covalentlybound to an albumin -binding moiety
  VARIANT 23: NOTE = X is Aib
  VARIANT 32: NOTE = X is Aib
  MOD_RES 38: NOTE = AMIDATION

SEQ ID NO: 90 - protein, 38 aa, synthetic construct; identical to SEQ ID NO: 62
  SOURCE 1..38
  MOD_RES 1: NOTE = ACETYLATION
  VARIANT 7: NOTE = D-valine
  MOD_RES 12: NOTE = the epsilon-amino group of the lysine side chain is covalentlybound to an albumin -binding moiety
  VARIANT 32: NOTE = X is 4-Pip
  MOD_RES 38: NOTE = AMIDATION

SEQ ID NO: 91 - protein, 38 aa, synthetic construct; identical to SEQ ID NO: 63
  SOURCE 1..38
  MOD_RES 1: NOTE = ACETYLATION
  VARIANT 7: NOTE = D-valine
  MOD_RES 12: NOTE = the epsilon-amino group of the lysine side chain is covalentlybound to an albumin -binding moiety
  VARIANT 23: NOTE = X is Aib
  VARIANT 32: NOTE = X is 4-Pip
  MOD_RES 38: NOTE = AMIDATION

SEQ ID NO: 92 - protein, 37 aa, synthetic construct; identical to SEQ ID NO: 33
  SOURCE 1..37
  MOD_RES 1: NOTE = ACETYLATION
  VARIANT 6: NOTE = D-valine
  MOD_RES 11: NOTE = the epsilon-amino group of the lysine side chain is covalentlybound to an albumin -binding moiety
  MOD_RES 37: NOTE = AMIDATION

SEQ ID NO: 93 - protein, 37 aa, synthetic construct; identical to SEQ ID NO: 33
  SOURCE 1..37
  VARIANT 6: NOTE = D-valine
  MOD_RES 11: NOTE = the epsilon-amino group of the lysine side chain is covalentlybound to an albumin -binding moiety
  MOD_RES 37: NOTE = AMIDATION

SEQ ID NO: 94 - protein, 37 aa, synthetic construct; identical to SEQ ID NO: 33
  SOURCE 1..37
  MOD_RES 1: NOTE = Acetylated with a propanoyl group
  MOD_RES 11: NOTE = the epsilon-amino group of the lysine side chain is covalentlybound to an albumin -binding moiety
  MOD_RES 37: NOTE = AMIDATION

SEQ ID NO: 95 - protein, 37 aa, synthetic construct; identical to SEQ ID NO: 33
  SOURCE 1..37
  MOD_RES 1: NOTE = Acetylated with a butanoyl group
  MOD_RES 11: NOTE = the epsilon-amino group of the lysine side chain is covalentlybound to an albumin -binding moiety
  MOD_RES 37: NOTE = AMIDATION

SEQ ID NO: 96 - protein, 37 aa, synthetic construct; identical to SEQ ID NO: 33
  SOURCE 1..37
  MOD_RES 1: NOTE = Acetylated with a pentanoyl group
  MOD_RES 11: NOTE = the epsilon-amino group of the lysine side chain is covalentlybound to an albumin -binding moiety
  MOD_RES 37: NOTE = AMIDATION

SEQ ID NO: 97 - protein, 38 aa, synthetic construct; identical to SEQ ID NO: 11
  SOURCE 1..38
  MOD_RES 1: NOTE = ACETYLATION
  MOD_RES 12: NOTE = the epsilon-amino group of the lysine side chain is covalentlybound to an albumin -binding moiety
  VARIANT 32: NOTE = X is Aib
  MOD_RES 38: NOTE = AMIDATION

SEQ ID NO: 98 - protein, 38 aa, synthetic construct; identical to SEQ ID NO: 11
  SOURCE 1..38
  MOD_RES 1: NOTE = ACETYLATION
  VARIANT 7: NOTE = D-valine
  MOD_RES 12: NOTE = the epsilon-amino group of the lysine side chain is covalentlybound to an albumin -binding moiety
  VARIANT 32: NOTE = X is Aib
  MOD_RES 38: NOTE = AMIDATION

SEQ ID NO: 99 - protein, 37 aa, synthetic construct; identical to SEQ ID NO: 45
  SOURCE 1..37
  MOD_RES 1: NOTE = ACETYLATION
  VARIANT 6: NOTE = D-valine
  MOD_RES 11: NOTE = the epsilon-amino group of the lysine side chain is covalentlybound to an albumin -binding moiety
  VARIANT 31: NOTE = X is Aib
  MOD_RES 37: NOTE = AMIDATION

SEQ ID NO: 100 - protein, 38 aa, synthetic construct; identical to SEQ ID NO: 47
  SOURCE 1..38
  MOD_RES 1: NOTE = ACETYLATION
  VARIANT 7: NOTE = D-valine
  MOD_RES 12: NOTE = the epsilon-amino group of the lysine side chain is covalentlybound to an albumin -binding moiety
  MOD_RES 38: NOTE = AMIDATION

SEQ ID NO: 101 - protein, 37 aa, synthetic construct
  SOURCE 1..37
  MOD_RES 1: NOTE = ACETYLATION
  VARIANT 6: NOTE = D-valine
  MOD_RES 11: NOTE = the epsilon-amino group of the lysine side chain is covalentlybound to an albumin -binding moiety
  MOD_RES 37: NOTE = AMIDATION
VLSLDVPIKLKKILLEQEKQKKQREQAETNAQILAQV

SEQ ID NO: 102 - protein, 38 aa, synthetic construct; identical to SEQ ID NO: 48
  SOURCE 1..38
  MOD_RES 1: NOTE = ACETYLATION
  MOD_RES 12: NOTE = the epsilon-amino group of the lysine side chain is covalentlybound to an albumin -binding moiety
  MOD_RES 38: NOTE = AMIDATION

SEQ ID NO: 103 - protein, 38 aa, synthetic construct; identical to SEQ ID NO: 48
  SOURCE 1..38
  MOD_RES 1: NOTE = ACETYLATION
  VARIANT 7: NOTE = D-valine
  MOD_RES 12: NOTE = the epsilon-amino group of the lysine side chain is covalentlybound to an albumin -binding moiety
  MOD_RES 38: NOTE = AMIDATION

SEQ ID NO: 104 - protein, 38 aa, synthetic construct; identical to SEQ ID NO: 11
  SOURCE 1..38
  MOD_RES 1: NOTE = ACETYLATION
  VARIANT 7: NOTE = D-valine
  MOD_RES 12: NOTE = the epsilon-amino group of the lysine side chain is covalentlybound to an albumin -binding moiety
  VARIANT 32: NOTE = X is Abu
  MOD_RES 38: NOTE = AMIDATION

SEQ ID NO: 105 - protein, 38 aa, synthetic construct; identical to SEQ ID NO: 11
  SOURCE 1..38
  MOD_RES 1: NOTE = ACETYLATION
  VARIANT 7: NOTE = D-valine
  MOD_RES 12: NOTE = the epsilon-amino group of the lysine side chain is covalentlybound to an albumin -binding moiety
  VARIANT 32: NOTE = X is Nva
  MOD_RES 38: NOTE = AMIDATION

SEQ ID NO: 106 - protein, 38 aa, synthetic construct; identical to SEQ ID NO: 11
  SOURCE 1..38
  MOD_RES 1: NOTE = ACETYLATION
  VARIANT 7: NOTE = D-valine
  MOD_RES 12: NOTE = the epsilon-amino group of the lysine side chain is covalentlybound to an albumin -binding moiety
  VARIANT 32: NOTE = X is alpha-methyl-leucine
  MOD_RES 38: NOTE = AMIDATION

SEQ ID NO: 107 - protein, 38 aa, synthetic construct; identical to SEQ ID NO: 11
  SOURCE 1..38
  MOD_RES 1: NOTE = ACETYLATION
  VARIANT 7: NOTE = D-valine
  MOD_RES 12: NOTE = the epsilon-amino group of the lysine side chain is covalentlybound to an albumin -binding moiety
  VARIANT 32: NOTE = X is Dap
  MOD_RES 38: NOTE = AMIDATION

SEQ ID NO: 108 - protein, 38 aa, synthetic construct; identical to SEQ ID NO: 56
  SOURCE 1..38
  MOD_RES 1: NOTE = ACETYLATION
  VARIANT 7: NOTE = D-valine
  MOD_RES 12: NOTE = the epsilon-amino group of the lysine side chain is covalentlybound to an albumin -binding moiety
  MOD_RES 38: NOTE = AMIDATION

SEQ ID NO: 109 - protein, 38 aa, synthetic construct; identical to SEQ ID NO: 11
  SOURCE 1..38
  MOD_RES 1: NOTE = ACETYLATION
  VARIANT 7: NOTE = D-valine
  MOD_RES 12: NOTE = the epsilon-amino group of the lysine side chain is covalentlybound to an albumin -binding moiety
  VARIANT 32: NOTE = X is 4-Pip
  MOD_RES 38: NOTE = AMIDATION

SEQ ID NO: 110 - protein, 38 aa, synthetic construct; identical to SEQ ID NO: 38
  SOURCE 1..38
  MOD_RES 1: NOTE = ACETYLATION
  VARIANT 7: NOTE = D-valine
  VARIANT 11: NOTE = X is alpha-methyl-leucine
  MOD_RES 12: NOTE = the epsilon-amino group of the lysine side chain is covalentlybound to an albumin -binding moiety
  VARIANT 32: NOTE = X is Aib
  MOD_RES 38: NOTE = AMIDATION

SEQ ID NO: 111 - protein, 38 aa, synthetic construct; identical to SEQ ID NO: 49
  SOURCE 1..38
  MOD_RES 1: NOTE = ACETYLATION
  VARIANT 7: NOTE = D-valine
  VARIANT 11: NOTE = X is alpha-methyl-leucine
  MOD_RES 12: NOTE = the epsilon-amino group of the lysine side chain is covalentlybound to an albumin -binding moiety
  MOD_RES 38: NOTE = AMIDATION

SEQ ID NO: 112 - protein, 38 aa, synthetic construct
  SOURCE 1..38
  MOD_RES 1: NOTE = ACETYLATION
  VARIANT 7: NOTE = D-valine
  VARIANT 11: NOTE = X is alpha-methyl-leucine
  MOD_RES 12: NOTE = the epsilon-amino group of the lysine side chain is covalentlybound to an albumin -binding moiety
  MOD_RES 38: NOTE = AMIDATION
IVLSLDVPIKXKKILLEQEKQKKQREQAETNAQILAQV

SEQ ID NO: 113 - protein, 38 aa, synthetic construct; identical to SEQ ID NO: 47
  SOURCE 1..38
  MOD_RES 1: NOTE = METHYLATION
  VARIANT 7: NOTE = D-valine
  MOD_RES 12: NOTE = the epsilon-amino group of the lysine side chain is covalentlybound to an albumin -binding moiety
  MOD_RES 38: NOTE = AMIDATION

SEQ ID NO: 114 - protein, 38 aa, synthetic construct; identical to SEQ ID NO: 11
  SOURCE 1..38
  MOD_RES 1: NOTE = METHYLATION
  VARIANT 7: NOTE = D-valine
  MOD_RES 12: NOTE = the epsilon-amino group of the lysine side chain is covalentlybound to an albumin -binding moiety
  VARIANT 32: NOTE = X is Abu
  MOD_RES 38: NOTE = AMIDATION

SEQ ID NO: 115 - protein, 38 aa, synthetic construct; identical to SEQ ID NO: 11
  SOURCE 1..38
  MOD_RES 1: NOTE = METHYLATION
  VARIANT 7: NOTE = D-valine
  MOD_RES 12: NOTE = the epsilon-amino group of the lysine side chain is covalentlybound to an albumin -binding moiety
  VARIANT 32: NOTE = X is Dap
  MOD_RES 38: NOTE = AMIDATION

SEQ ID NO: 116 - protein, 38 aa, synthetic construct; identical to SEQ ID NO: 56
  SOURCE 1..38
  MOD_RES 1: NOTE = METHYLATION
  VARIANT 7: NOTE = D-valine
  MOD_RES 12: NOTE = the epsilon-amino group of the lysine side chain is covalentlybound to an albumin -binding moiety
  MOD_RES 38: NOTE = AMIDATION

SEQ ID NO: 117 - protein, 38 aa, synthetic construct; identical to SEQ ID NO: 11
  SOURCE 1..38
  MOD_RES 1: NOTE = METHYLATION
  VARIANT 7: NOTE = D-valine
  MOD_RES 12: NOTE = the epsilon-amino group of the lysine side chain is covalentlybound to an albumin -binding moiety
  VARIANT 32: NOTE = X is 4-Pip
  MOD_RES 38: NOTE = AMIDATION

SEQ ID NO: 118 - protein, 38 aa, synthetic construct; identical to SEQ ID NO: 11
  SOURCE 1..38
  MOD_RES 1: NOTE = METHYLATION
  VARIANT 7: NOTE = D-valine
  MOD_RES 12: NOTE = the epsilon-amino group of the lysine side chain is covalentlybound to an albumin -binding moiety
  VARIANT 32: NOTE = X is Aib
  MOD_RES 38: NOTE = AMIDATION

SEQ ID NO: 119 - protein, 38 aa, synthetic construct; identical to SEQ ID NO: 38
  SOURCE 1..38
  MOD_RES 1: NOTE = METHYLATION
  VARIANT 7: NOTE = D-valine
  VARIANT 11: NOTE = X is alpha-methyl-leucine
  MOD_RES 12: NOTE = the epsilon-amino group of the lysine side chain is covalentlybound to an albumin -binding moiety
  VARIANT 32: NOTE = X is Aib
  MOD_RES 38: NOTE = AMIDATION

SEQ ID NO: 120 - protein, 37 aa, synthetic construct; identical to SEQ ID NO: 45
  SOURCE 1..37
  MOD_RES 1: NOTE = Acetylated with a pentanoyl group
  VARIANT 6: NOTE = D-valine
  MOD_RES 11: NOTE = the epsilon-amino group of the lysine side chain is covalentlybound to an albumin -binding moiety
  VARIANT 31: NOTE = X is Aib
  MOD_RES 37: NOTE = AMIDATION

SEQ ID NO: 121 - protein, 37 aa, synthetic construct; identical to SEQ ID NO: 81
  SOURCE 1..37
  MOD_RES 1: NOTE = Acetylated with a pentanoyl group
  VARIANT 6: NOTE = D-valine
  MOD_RES 11: NOTE = the epsilon-amino group of the lysine side chain is covalentlybound to an albumin -binding moiety
  MOD_RES 37: NOTE = AMIDATION

SEQ ID NO: 122 - protein, 37 aa, synthetic construct; identical to SEQ ID NO: 101
  SOURCE 1..37
  MOD_RES 1: NOTE = Acetylated with a pentanoyl group
  VARIANT 6: NOTE = D-valine
  MOD_RES 11: NOTE = the epsilon-amino group of the lysine side chain is covalentlybound to an albumin -binding moiety
  MOD_RES 37: NOTE = AMIDATION

SEQ ID NO: 123 - protein, 37 aa, synthetic construct; identical to SEQ ID NO: 46
  SOURCE 1..37
  MOD_RES 1: NOTE = Acetylated with a pentanoyl group
  VARIANT 5: NOTE = D-valine
  VARIANT 10: NOTE = X is alpha-methyl-leucine
  MOD_RES 11: NOTE = the epsilon-amino group of the lysine side chain is covalentlybound to an albumin -binding moiety
  VARIANT 31: NOTE = X is Aib
  MOD_RES 37: NOTE = AMIDATION

SEQ ID NO: 124 - protein, 37 aa, synthetic construct
  SOURCE 1..37
  MOD_RES 1: NOTE = Acetylated with a pentanoyl group
  VARIANT 7: NOTE = D-valine
  VARIANT 10: NOTE = X is alpha-methyl-leucine
  MOD_RES 11: NOTE = the epsilon-amino group of the lysine side chain is covalentlybound to an albumin -binding moiety
  MOD_RES 37: NOTE = AMIDATION
VLSLDVPIKXKKILLEQEKQKKQREQAETNVQILAQV

SEQ ID NO: 125 - protein, 38 aa, synthetic construct; identical to SEQ ID NO: 11
  SOURCE 1..38
  MOD_RES 1: NOTE = ACETYLATION
  VARIANT 7: NOTE = D-valine
  MOD_RES 12: NOTE = the epsilon-amino group of the lysine side chain is covalentlybound to an albumin -binding moiety
  VARIANT 32: NOTE = X is Aib
  MOD_RES 38: NOTE = AMIDATION

SEQ ID NO: 126 - protein, 38 aa, synthetic construct; identical to SEQ ID NO: 47
  SOURCE 1..38
  MOD_RES 1: NOTE = ACETYLATION
  VARIANT 7: NOTE = D-valine
  MOD_RES 12: NOTE = the epsilon-amino group of the lysine side chain is covalentlybound to an albumin -binding moiety
  MOD_RES 38: NOTE = AMIDATION

SEQ ID NO: 127 - protein, 38 aa, synthetic construct; identical to SEQ ID NO: 11
  SOURCE 1..38
  MOD_RES 1: NOTE = ACETYLATION
  VARIANT 7: NOTE = D-valine
  MOD_RES 12: NOTE = the epsilon-amino group of the lysine side chain is covalentlybound to an albumin -binding moiety
  VARIANT 32: NOTE = X is Abu
  MOD_RES 38: NOTE = AMIDATION

SEQ ID NO: 128 - protein, 38 aa, synthetic construct; identical to SEQ ID NO: 11
  SOURCE 1..38
  MOD_RES 1: NOTE = ACETYLATION
  VARIANT 7: NOTE = D-valine
  MOD_RES 12: NOTE = the epsilon-amino group of the lysine side chain is covalentlybound to an albumin -binding moiety
  VARIANT 32: NOTE = X is Dap
  MOD_RES 38: NOTE = AMIDATION

SEQ ID NO: 129 - protein, 38 aa, synthetic construct; identical to SEQ ID NO: 11
  SOURCE 1..38
  MOD_RES 1: NOTE = ACETYLATION
  VARIANT 7: NOTE = D-valine
  MOD_RES 12: NOTE = the epsilon-amino group of the lysine side chain is covalentlybound to an albumin -binding moiety
  VARIANT 32: NOTE = X is 4-Pip
  MOD_RES 38: NOTE = AMIDATION

SEQ ID NO: 130 - protein, 38 aa, synthetic construct; identical to SEQ ID NO: 56
  SOURCE 1..38
  MOD_RES 1: NOTE = ACETYLATION
  VARIANT 7: NOTE = D-valine
  MOD_RES 12: NOTE = the epsilon-amino group of the lysine side chain is covalentlybound to an albumin -binding moiety
  MOD_RES 38: NOTE = AMIDATION

SEQ ID NO: 131 - protein, 38 aa, synthetic construct; identical to SEQ ID NO: 62
  SOURCE 1..38
  MOD_RES 1: NOTE = ACETYLATION
  VARIANT 7: NOTE = D-valine
  MOD_RES 12: NOTE = the epsilon-amino group of the lysine side chain is covalentlybound to an albumin -binding moiety
  VARIANT 32: NOTE = X is 4-Pip
  MOD_RES 38: NOTE = AMIDATION

SEQ ID NO: 132 - protein, 38 aa, synthetic construct; identical to SEQ ID NO: 63
  SOURCE 1..38
  MOD_RES 1: NOTE = ACETYLATION
  VARIANT 7: NOTE = D-valine
  MOD_RES 12: NOTE = the epsilon-amino group of the lysine side chain is covalentlybound to an albumin -binding moiety
  VARIANT 23: NOTE = X is Aib
  VARIANT 32: NOTE = X is 4-Pip
  MOD_RES 38: NOTE = AMIDATION

SEQ ID NO: 133 - protein, 38 aa, synthetic construct; identical to SEQ ID NO: 11
  SOURCE 1..38
  MOD_RES 1: NOTE = ACETYLATION
  VARIANT 7: NOTE = D-valine
  MOD_RES 12: NOTE = the epsilon-amino group of the lysine side chain is covalentlybound to an albumin -binding moiety
  VARIANT 32: NOTE = X is Thp
  MOD_RES 38: NOTE = AMIDATION

SEQ ID NO: 134 - protein, 38 aa, synthetic construct; identical to SEQ ID NO: 11
  SOURCE 1..38
  MOD_RES 1: NOTE = ACETYLATION
  VARIANT 7: NOTE = D-valine
  MOD_RES 12: NOTE = the epsilon-amino group of the lysine side chain is covalentlybound to an albumin -binding moiety
  VARIANT 32: NOTE = X is Chx
  MOD_RES 38: NOTE = AMIDATION

SEQ ID NO: 135 - protein, 38 aa, synthetic construct; identical to SEQ ID NO: 11
  SOURCE 1..38
  MOD_RES 1: NOTE = ACETYLATION
  VARIANT 7: NOTE = D-valine
  MOD_RES 12: NOTE = the epsilon-amino group of the lysine side chain is covalentlybound to an albumin -binding moiety
  VARIANT 32: NOTE = X is Cpex
  MOD_RES 38: NOTE = AMIDATION

SEQ ID NO: 136 - protein, 38 aa, synthetic construct; identical to SEQ ID NO: 11
  SOURCE 1..38
  MOD_RES 1: NOTE = ACETYLATION
  VARIANT 7: NOTE = D-valine
  MOD_RES 12: NOTE = the epsilon-amino group of the lysine side chain is covalentlybound to an albumin -binding moiety
  VARIANT 32: NOTE = X is Cpx
  MOD_RES 38: NOTE = AMIDATION

SEQ ID NO: 137 - protein, 38 aa, synthetic construct; identical to SEQ ID NO: 11
  SOURCE 1..38
  MOD_RES 1: NOTE = METHYLATION
  VARIANT 7: NOTE = D-valine
  MOD_RES 12: NOTE = the epsilon-amino group of the lysine side chain is covalentlybound to an albumin -binding moiety
  VARIANT 32: NOTE = X is Aib
  MOD_RES 38: NOTE = AMIDATION

SEQ ID NO: 138 - protein, 38 aa, synthetic construct; identical to SEQ ID NO: 47
  SOURCE 1..38
  MOD_RES 1: NOTE = METHYLATION
  VARIANT 7: NOTE = D-valine
  MOD_RES 12: NOTE = the epsilon-amino group of the lysine side chain is covalentlybound to an albumin -binding moiety
  MOD_RES 38: NOTE = AMIDATION

SEQ ID NO: 139 - protein, 38 aa, synthetic construct; identical to SEQ ID NO: 11
  SOURCE 1..38
  MOD_RES 1: NOTE = METHYLATION
  VARIANT 7: NOTE = D-valine
  MOD_RES 12: NOTE = the epsilon-amino group of the lysine side chain is covalentlybound to an albumin -binding moiety
  VARIANT 32: NOTE = X is Abu
  MOD_RES 38: NOTE = AMIDATION

SEQ ID NO: 140 - protein, 38 aa, synthetic construct; identical to SEQ ID NO: 11
  SOURCE 1..38
  MOD_RES 1: NOTE = METHYLATION
  VARIANT 7: NOTE = D-valine
  MOD_RES 12: NOTE = the epsilon-amino group of the lysine side chain is covalentlybound to an albumin -binding moiety
  VARIANT 32: NOTE = X is Dap
  MOD_RES 38: NOTE = AMIDATION

SEQ ID NO: 141 - protein, 38 aa, synthetic construct; identical to SEQ ID NO: 11
  SOURCE 1..38
  MOD_RES 1: NOTE = METHYLATION
  VARIANT 7: NOTE = D-valine
  MOD_RES 12: NOTE = the epsilon-amino group of the lysine side chain is covalentlybound to an albumin -binding moiety
  VARIANT 32: NOTE = X is 4-Pip
  MOD_RES 38: NOTE = AMIDATION

SEQ ID NO: 142 - protein, 38 aa, synthetic construct; identical to SEQ ID NO: 56
  SOURCE 1..38
  MOD_RES 1: NOTE = METHYLATION
  VARIANT 7: NOTE = D-valine
  MOD_RES 12: NOTE = the epsilon-amino group of the lysine side chain is covalentlybound to an albumin -binding moiety
  MOD_RES 38: NOTE = AMIDATION

SEQ ID NO: 143 - protein, 38 aa, synthetic construct; identical to SEQ ID NO: 11
  SOURCE 1..38
  MOD_RES 1: NOTE = METHYLATION
  VARIANT 7: NOTE = D-valine
  MOD_RES 12: NOTE = the epsilon-amino group of the lysine side chain is covalentlybound to an albumin -binding moiety
  VARIANT 32: NOTE = X is Thp
  MOD_RES 38: NOTE = AMIDATION

SEQ ID NO: 144 - protein, 38 aa, synthetic construct; identical to SEQ ID NO: 62
  SOURCE 1..38
  MOD_RES 1: NOTE = METHYLATION
  VARIANT 7: NOTE = D-valine
  MOD_RES 12: NOTE = the epsilon-amino group of the lysine side chain is covalentlybound to an albumin -binding moiety
  VARIANT 32: NOTE = X is Aib
  MOD_RES 38: NOTE = AMIDATION

SEQ ID NO: 145 - protein, 38 aa, synthetic construct; identical to SEQ ID NO: 63
  SOURCE 1..38
  MOD_RES 1: NOTE = METHYLATION
  VARIANT 7: NOTE = D-valine
  MOD_RES 12: NOTE = the epsilon-amino group of the lysine side chain is covalentlybound to an albumin -binding moiety
  VARIANT 23: NOTE = X is Aib
  VARIANT 32: NOTE = X is Aib
  MOD_RES 38: NOTE = AMIDATION

SEQ ID NO: 146 - protein, 38 aa, synthetic construct
  SOURCE 1..38
  REGION 1..38: NOTE = Comp 3
  VARIANT 7: NOTE = D-valine
  MOD_RES 12: NOTE = the epsilon-amino group of the lysine side chain is covalentlybound to an albumin -binding moiety
  MOD_RES 38: NOTE = AMIDATION
IVLSLDVPIKLKQILLKQERQKKQREQAEKNKQILEQV

SEQ ID NO: 147 - protein, 38 aa, synthetic construct; identical to SEQ ID NO: 146
  SOURCE 1..38
  REGION 1..38: NOTE = Comp 2
  VARIANT 7: NOTE = D-valine
  MOD_RES 12: NOTE = the epsilon-amino group of the lysine side chain is covalentlybound to an albumin -binding moiety
  MOD_RES 38: NOTE = AMIDATION

SEQ ID NO: 148 - protein, 38 aa, synthetic construct; identical to SEQ ID NO: 146
  SOURCE 1..38
  VARIANT 7: NOTE = D-valine
  MOD_RES 12: NOTE = the epsilon-amino group of the lysine side chain is covalentlybound to an albumin -binding moiety
  MOD_RES 38: NOTE = AMIDATION

SEQ ID NO: 149 - protein, 38 aa, synthetic construct
  SOURCE 1..38
  VARIANT 7: NOTE = D-valine
  MOD_RES 12: NOTE = the epsilon-amino group of the lysine side chain is covalentlybound to an albumin -binding moiety
  MOD_RES 38: NOTE = AMIDATION
IVLSLDVPIKLKKILLEQEKQKKQREQAETNKQILAQV

SEQ ID NO: 150 - protein, 38 aa, synthetic construct; identical to SEQ ID NO: 146
  SOURCE 1..38
  VARIANT 7: NOTE = D-valine
  MOD_RES 12: NOTE = the epsilon-amino group of the lysine side chain is covalentlybound to an albumin -binding moiety
  MOD_RES 38: NOTE = AMIDATION

SEQ ID NO: 151 - protein, 38 aa, synthetic construct; identical to SEQ ID NO: 146
  VARIANT 7: NOTE = D-valine
  MOD_RES 12: NOTE = the epsilon-amino group of the lysine side chain is covalentlybound to an albumin -binding moiety
  MOD_RES 38: NOTE = AMIDATION
  SOURCE 1..38

SEQ ID NO: 152 - protein, 38 aa, synthetic construct; identical to SEQ ID NO: 62
  SOURCE 1..38
  MOD_RES 1: NOTE = Acetylated
  VARIANT 7: NOTE = D-Valine
  MOD_RES 12: NOTE = Lysine is bound to an albumine-binding moiety
  VARIANT 32: NOTE = X = 4-Pip
  MOD_RES 38: NOTE = Amidation

SEQ ID NO: 153 - protein, 38 aa, synthetic construct; identical to SEQ ID NO: 63
  SOURCE 1..38
  MOD_RES 1: NOTE = Acetylated
  VARIANT 7: NOTE = D-Valine
  MOD_RES 12: NOTE = Lysine is bound to an albumine-binding moiety
  VARIANT 23: NOTE = X = Aib
  VARIANT 32: NOTE = X = 4-Pip
  MOD_RES 38: NOTE = AMIDATION

SEQ ID NO: 154 - protein, 38 aa, synthetic construct; identical to SEQ ID NO: 62
  SOURCE 1..38
  MOD_RES 1: NOTE = N-Methylated
  VARIANT 7: NOTE = D-Valine
  VARIANT 32: NOTE = X = 4-Pip
  MOD_RES 38: NOTE = Amidation
  MOD_RES 12: NOTE = Lisine is bound to an albumin binding moiety

SEQ ID NO: 155 - protein, 38 aa, synthetic construct; identical to SEQ ID NO: 63
  SOURCE 1..38
  MOD_RES 1: NOTE = N-Methylated
  VARIANT 23: NOTE = X = Aib
  VARIANT 32: NOTE = X = 4-Pip
  MOD_RES 38: NOTE = Amidation
  VARIANT 7: NOTE = D-Valine
  MOD_RES 12: NOTE = Lysine is bound to an albumin binding moiety

SEQ ID NO: 156 - protein, 37 aa, synthetic construct; identical to SEQ ID NO: 45
  SOURCE 1..37
  MOD_RES 1: NOTE = Acylated with Hexanoyl
  VARIANT 6: NOTE = D-Valine
  VARIANT 31: NOTE = X = Aib
  MOD_RES 37: NOTE = Amidation
  MOD_RES 11: NOTE = Lysine is bound to an albumin binding moiety

SEQ ID NO: 157 - protein, 37 aa, synthetic construct; identical to SEQ ID NO: 45
  SOURCE 1..37
  MOD_RES 1: NOTE = Acylated with Hexanoyl
  VARIANT 6: NOTE = D-Valine
  VARIANT 31: NOTE = X = 4-Pip
  MOD_RES 37: NOTE = Amidation
  MOD_RES 11: NOTE = Lysine is bound to an albumin binding moiety

SEQ ID NO: 158 - protein, 37 aa, synthetic construct; identical to SEQ ID NO: 45
  SOURCE 1..37
  MOD_RES 1: NOTE = Acylation with Decanoyl
  VARIANT 6: NOTE = D-Valine
  MOD_RES 11: NOTE = Lysine is bound to an albumin binding moiety
  VARIANT 31: NOTE = X = Aib
  MOD_RES 37: NOTE = Amidation

SEQ ID NO: 159 - protein, 37 aa, synthetic construct; identical to SEQ ID NO: 45
  SOURCE 1..37
  MOD_RES 1: NOTE = N-Methylated
  VARIANT 6: NOTE = D-Valine
  MOD_RES 11: NOTE = Lysine is bound to an albumin binding moiety
  VARIANT 31: NOTE = X = Aib
  MOD_RES 37: NOTE = amidation

SEQ ID NO: 160 - protein, 37 aa, synthetic construct; identical to SEQ ID NO: 45
  SOURCE 1..37
  MOD_RES 1: NOTE = N-Methylated
  VARIANT 6: NOTE = D-Valine
  MOD_RES 11: NOTE = Lysine is bound to an albumin binding moiety
  VARIANT 31: NOTE = X = 4-Pip
  MOD_RES 37: NOTE = amidation

SEQ ID NO: 161 - protein, 38 aa, synthetic construct; identical to SEQ ID NO: 62
  SOURCE 1..38
  MOD_RES 1: NOTE = Acetylated
  VARIANT 7: NOTE = D-Valine
  VARIANT 32: NOTE = X = Aib
  MOD_RES 38: NOTE; NOTE = Amidation
  MOD_RES 12: NOTE; NOTE = Lysine side chain is bound to an albumin-binding moiety

SEQ ID NO: 162 - protein, 38 aa, synthetic construct; identical to SEQ ID NO: 63
  SOURCE 1..38
  MOD_RES 1: NOTE = Acetylated
  VARIANT 7: NOTE = D-Valine
  MOD_RES 12: NOTE = Lysine is bound to an albumin binding moiety
  VARIANT 23: NOTE = X = Aib
  VARIANT 32: NOTE = X = Aib
  MOD_RES 38: NOTE = Amidation

SEQ ID NO: 163 - protein, 38 aa, synthetic construct
  SOURCE 1..38
  MOD_RES 1: NOTE = acetylation
  VARIANT 7: NOTE = D-Valine
  MOD_RES 12: NOTE = Lysine is bound to an albumin binding moiety
  VARIANT 32: NOTE = X = Aib
  MOD_RES 38: NOTE = amidation
IVLSLDVPIALKKILLEQEKQKKQREQAETNXQILAQV

SEQ ID NO: 164 - protein, 38 aa, synthetic construct
  SOURCE 1..38
  MOD_RES 1: NOTE = Acetylated
  VARIANT 7: NOTE = D-Valine
  MOD_RES 12: NOTE = Lysine is bound to an albumin binding moiety
  VARIANT 32: NOTE = X = Aib
  MOD_RES 38: NOTE = Amidation
IVLSLDVPIKLKAILLEQEKQKKQREQAETNXQILAQV

SEQ ID NO: 165 - protein, 38 aa, synthetic construct
  SOURCE 1..38
  MOD_RES 1: NOTE = Acetylated
  VARIANT 7: NOTE = D-Valine
  MOD_RES 12: NOTE = Lysine is bound to an albumin binding moiety
  VARIANT 32: NOTE = X = Aib
  MOD_RES 38: NOTE = amidation
IVLSLDVPIKLKKILLEQEAQKKQREQAETNXQILAQV

SEQ ID NO: 166 - protein, 38 aa, synthetic construct
  SOURCE 1..38
  MOD_RES 1: NOTE = acetylation
  VARIANT 7: NOTE = D-Valine
  MOD_RES 12: NOTE = Lysine is bound to an albumin binding moiety
  VARIANT 32: NOTE = X = Aib
  MOD_RES 38: NOTE = amidation
IVLSLDVPIKLKKILLEQEKQAKQREQAETNXQILAQV

SEQ ID NO: 167 - protein, 38 aa, synthetic construct
  SOURCE 1..38
  MOD_RES 1: NOTE = acetylation
  VARIANT 7: NOTE = D-Valine
  MOD_RES 12: NOTE = Lysine is bound to an albumin binding moiety
  VARIANT 32: NOTE = X = Aib
  MOD_RES 38: NOTE = Amidation
IVLSLDVPIKLKKILLEQEKQKKQAEQAETNXQILAQV

SEQ ID NO: 168 - protein, 38 aa, synthetic construct
  SOURCE 1..38
  MOD_RES 1: NOTE = Acetylation
  VARIANT 7: NOTE = D-Valine
  MOD_RES 12: NOTE = Lysine is bound to an albumin binding moiety
  VARIANT 32: NOTE = X = Aib
  MOD_RES 38: NOTE = Amidation
IVLSLDVPIKLKKILLEQEKQKEQREQAETNXQILAQV

SEQ ID NO: 169 - protein, 38 aa, synthetic construct; identical to SEQ ID NO: 62
  SOURCE 1..38
  MOD_RES 1: NOTE = Acetylation
  VARIANT 7: NOTE = D-Valine
  MOD_RES 12: NOTE = Lysine is bound to an albumin binding moiety
  VARIANT 32: NOTE = X = 4-Pip
  MOD_RES 38: NOTE = amidation

SEQ ID NO: 170 - protein, 38 aa, synthetic construct; identical to SEQ ID NO: 63
  SOURCE 1..38
  MOD_RES 1: NOTE = acetylation
  VARIANT 7: NOTE = D-Valine
  MOD_RES 12: NOTE = Lysine is bound to an albumin binding moiety
  VARIANT 23: NOTE = X = Aib
  VARIANT 32: NOTE = X = 4-Pip
  MOD_RES 38: NOTE = amidation

SEQ ID NO: 171 - protein, 38 aa, synthetic construct; identical to SEQ ID NO: 11
  SOURCE 1..38
  MOD_RES 1: NOTE = acetylated
  VARIANT 7: NOTE = D-Valine
  MOD_RES 12: NOTE = Lysine is bound to an albumin binding moiety
  VARIANT 32: NOTE = X = Aib
  MOD_RES 38: NOTE = Amidation

SEQ ID NO: 172 - protein, 38 aa, synthetic construct; identical to SEQ ID NO: 11
  SOURCE 1..38
  MOD_RES 1: NOTE = Acetylated
  VARIANT 7: NOTE = D-Valine
  MOD_RES 12: NOTE = Lysine is bound to an albumin binding moiety
  VARIANT 32: NOTE = X = 4-Pip
  MOD_RES 38: NOTE = amidation

SEQ ID NO: 173 - protein, 38 aa, synthetic construct; identical to SEQ ID NO: 63
  SOURCE 1..38
  MOD_RES 1: NOTE = acetylation
  VARIANT 7: NOTE = D-Valine
  MOD_RES 12: NOTE = Lysine is bound to an albumin binding moiety
  VARIANT 23: NOTE = X = Aib
  VARIANT 32: NOTE = X = 4-Pip
  MOD_RES 38: NOTE = amidation

SEQ ID NO: 174 - protein, 38 aa, synthetic construct; identical to SEQ ID NO: 11
  SOURCE 1..38
  MOD_RES 1: NOTE = acetylation
  VARIANT 7: NOTE = D-Valine
  MOD_RES 12: NOTE = Lysine is bound to an albumin binding moeity
  VARIANT 32: NOTE = X = Aib
  MOD_RES 38: NOTE = amidation

SEQ ID NO: 175 - protein, 38 aa, synthetic construct; identical to SEQ ID NO: 11
  SOURCE 1..38
  MOD_RES 1: NOTE = acetylation
  VARIANT 7: NOTE = D-Valine
  MOD_RES 12: NOTE = Lysine is bound to an albumin binding moiety
  VARIANT 32: NOTE = X = 4-Pip
  MOD_RES 38: NOTE = amidation

SEQ ID NO: 176 - protein, 38 aa, synthetic construct; identical to SEQ ID NO: 62
  SOURCE 1..38
  MOD_RES 1: NOTE = N-Methylated
  VARIANT 7: NOTE = D-Valine
  MOD_RES 12: NOTE = Lysine is bound to an albumin binding moiety
  VARIANT 32: NOTE = X = Aib
  MOD_RES 38: NOTE = Amidation

SEQ ID NO: 177 - protein, 38 aa, synthetic construct; identical to SEQ ID NO: 63
  SOURCE 1..38
  MOD_RES 1: NOTE = N-Methylated
  VARIANT 7: NOTE = D-Valine
  MOD_RES 12: NOTE = Lysine is bound to an albumin binding moiety
  VARIANT 23: NOTE = X = Aib
  VARIANT 32: NOTE = X = Aib
  MOD_RES 38: NOTE = amidation

SEQ ID NO: 178 - protein, 38 aa, synthetic construct; identical to SEQ ID NO: 11
  SOURCE 1..38
  MOD_RES 1: NOTE = N-Methylated
  VARIANT 7: NOTE = D-Valine
  MOD_RES 12: NOTE = Lysine is bound to an albumin binding moiety
  VARIANT 32: NOTE = X = Aib
  MOD_RES 38: NOTE = amidation

SEQ ID NO: 179 - protein, 38 aa, synthetic construct; identical to SEQ ID NO: 11
  SOURCE 1..38
  MOD_RES 1: NOTE = N-Methylated
  VARIANT 7: NOTE = D-Valine
  MOD_RES 12: NOTE = Lysine is bound to an albumin binding moiety
  VARIANT 32: NOTE = X = Aib
  MOD_RES 38: NOTE = amidation

SEQ ID NO: 180 - protein, 37 aa, synthetic construct; identical to SEQ ID NO: 45
  SOURCE 1..37
  MOD_RES 1: NOTE = Acylation with Pentanoyl
  VARIANT 6: NOTE = D-Valine
  MOD_RES 11: NOTE = Lysine is bound to an albulin binding moiety
  VARIANT 31: NOTE = X = Aib
  MOD_RES 37: NOTE = Amidation

SEQ ID NO: 181 - protein, 37 aa, synthetic construct; identical to SEQ ID NO: 45
  SOURCE 1..37
  MOD_RES 1: NOTE = Acylation with Pentanoyl
  VARIANT 6: NOTE = D-Valine
  MOD_RES 11: NOTE = Lysine is bound to an albumin binding moiety
  VARIANT 31: NOTE = X = Aib
  MOD_RES 37: NOTE = amidation

SEQ ID NO: 182 - protein, 38 aa, synthetic construct; identical to SEQ ID NO: 11
  SOURCE 1..38
  MOD_RES 1: NOTE = Acetylation
  VARIANT 7: NOTE = D-Valine
  MOD_RES 12: NOTE = Lysine is bound to an albumin binding moiety
  VARIANT 32: NOTE = X = Aib
  MOD_RES 38: NOTE = amidation

SEQ ID NO: 183 - protein, 38 aa, synthetic construct; identical to SEQ ID NO: 11
  SOURCE 1..38
  MOD_RES 1: NOTE = Acetylation
  VARIANT 7: NOTE = D-Valine
  MOD_RES 12: NOTE = Lysine is bound to an albumin binding moiety
  VARIANT 32: NOTE = X = 4-Pip
  MOD_RES 38: NOTE = Amidation

SEQ ID NO: 184 - protein, 38 aa, synthetic construct; identical to SEQ ID NO: 63
  SOURCE 1..38
  MOD_RES 1: NOTE = Acetylation
  VARIANT 7: NOTE = D-Valine
  MOD_RES 12: NOTE = Lysine is bound to an albumin binding moiety
  VARIANT 23: NOTE = X = Aib
  VARIANT 32: NOTE = X = 4-Pip
  MOD_RES 38: NOTE = Amidation

SEQ ID NO: 185 - protein, 37 aa, synthetic construct; identical to SEQ ID NO: 45
  SOURCE 1..37
  MOD_RES 1: NOTE = Acylation with Pentanoyl
  VARIANT 6: NOTE = D-Valine
  MOD_RES 11: NOTE = Lysine is bound to an albumin binding moiety
  VARIANT 31: NOTE = X = Aib
  MOD_RES 37: NOTE = Amidation

SEQ ID NO: 186 - protein, 38 aa, synthetic construct; identical to SEQ ID NO: 11
  SOURCE 1..38
  MOD_RES 1: NOTE = N-Methylated
  VARIANT 7: NOTE = D-Valine
  MOD_RES 12: NOTE = Lysine is bound to an albumin binding moiety
  VARIANT 32: NOTE = X = Aib
  MOD_RES 38: NOTE = Amidation

SEQ ID NO: 187 - protein, 38 aa, synthetic construct; identical to SEQ ID NO: 62
  SOURCE 1..38
  MOD_RES 1: NOTE = Acetylation
  VARIANT 7: NOTE = D-Valine
  MOD_RES 12: NOTE = Lysine is bound to an albumin binding moiety
  VARIANT 32: NOTE = 4-Pip
  MOD_RES 38: NOTE = Amidation

SEQ ID NO: 188 - protein, 38 aa, synthetic construct; identical to SEQ ID NO: 63
  SOURCE 1..38
  MOD_RES 1: NOTE = Acetylation
  VARIANT 7: NOTE = D-Valine
  MOD_RES 12: NOTE = Lysine is bound to an albumin binding moiety
  VARIANT 23: NOTE = X = Aib
  VARIANT 32: NOTE = X = 4-Pip
  MOD_RES 38: NOTE = Amidation

SEQ ID NO: 189 - protein, 38 aa, synthetic construct; identical to SEQ ID NO: 62
  SOURCE 1..38
  MOD_RES 1: NOTE = Acetylation
  VARIANT 7: NOTE = D-Valine
  MOD_RES 12: NOTE = Lysine is bound to an albumin binding moiety
  VARIANT 32: NOTE = X = Aib
  MOD_RES 38: NOTE = Amidation

SEQ ID NO: 190 - protein, 38 aa, synthetic construct; identical to SEQ ID NO: 63
  SOURCE 1..38
  MOD_RES 1: NOTE = Acetylation
  VARIANT 7: NOTE = D-Valine
  MOD_RES 12: NOTE = Lysine is bound to an albumin binding moiety
  VARIANT 23: NOTE = X = Aib
  VARIANT 32: NOTE = X = Aib
  MOD_RES 38: NOTE = Amidation

SEQ ID NO: 191 - protein, 38 aa, synthetic construct
  SOURCE 1..38
  MOD_RES 1: NOTE = Acetylated
  VARIANT 7: NOTE = D-Valine
  MOD_RES 12: NOTE = Lysine is bound to an albumin binding moiety
  VARIANT 32: NOTE = X = Aib
  MOD_RES 38: NOTE = Amidation
IVLSLDVPIGLKKILLEQEKQKKQREQAETNXQILAQV

SEQ ID NO: 192 - protein, 38 aa, synthetic construct; identical to SEQ ID NO: 191
  SOURCE 1..38
  MOD_RES 1: NOTE = N-Methylated
  VARIANT 7: NOTE = D-Valine
  MOD_RES 12: NOTE = Lysine is bound to an albumin binding moiety
  VARIANT 32: NOTE = X = Aib
  MOD_RES 38: NOTE = amidation

SEQ ID NO: 193 - protein, 37 aa, synthetic construct; identical to SEQ ID NO: 45
  SOURCE 1..37
  MOD_RES 1: NOTE = Acylation with Pentanoyl
  VARIANT 6: NOTE = D-Valine
  MOD_RES 11: NOTE = Lysine is bound to an albumin binding moiety
  VARIANT 31: NOTE = X = Aib
  MOD_RES 37: NOTE = Amidation

SEQ ID NO: 194 - protein, 37 aa, synthetic construct; identical to SEQ ID NO: 15
  SOURCE 1..37
  MOD_RES 1: NOTE = Acylation with Pentanoyl
  VARIANT 6: NOTE = D-Valine
  MOD_RES 11: NOTE = Lysine is bound to an albumin binding moiety
  VARIANT 31: NOTE = X = Aib
  MOD_RES 37: NOTE = Amidation

SEQ ID NO: 195 - protein, 37 aa, synthetic construct
  SOURCE 1..37
  MOD_RES 1: NOTE = Acylation with Pentanoyl
  VARIANT 6: NOTE = D-Valine
  MOD_RES 11: NOTE = Lysine is bound to an albumin binding moiety
  VARIANT 31: NOTE = X = Aib
  MOD_RES 37: NOTE = Amidation
VLSLDVPIGLKKILLEQEKQKKQREQAETNXQILAQV

SEQ ID NO: 196 - protein, 38 aa, synthetic construct; identical to SEQ ID NO: 63
  SOURCE 1..38
  MOD_RES 1: NOTE = Acetylation
  VARIANT 7: NOTE = D-Valine
  MOD_RES 12: NOTE = Lysine is bound to an albulin binding moiety
  VARIANT 23: NOTE = X = Aib
  VARIANT 32: NOTE = X = 4-Pip
  MOD_RES 38: NOTE = Amidation

SEQ ID NO: 197 - protein, 38 aa, synthetic construct; identical to SEQ ID NO: 63
  SOURCE 1..38
  MOD_RES 1: NOTE = Acetylation
  VARIANT 7: NOTE = D-Valine
  MOD_RES 12: NOTE = Lysine is bound to an albumin binding moiety
  VARIANT 23: NOTE = X = Aib
  VARIANT 32: NOTE = X = Aib
  MOD_RES 38: NOTE = Amidation

SEQ ID NO: 198 - protein, 38 aa, synthetic construct; identical to SEQ ID NO: 11
  SOURCE 1..38
  MOD_RES 1: NOTE = Acetylation
  VARIANT 7: NOTE = D-Valine
  MOD_RES 12: NOTE = Lysine is bound to an albumin binding moiety
  VARIANT 32: NOTE = X = Thp
  MOD_RES 38: NOTE = amidation

SEQ ID NO: 199 - protein, 38 aa, synthetic construct; identical to SEQ ID NO: 11
  SOURCE 1..38
  MOD_RES 1: NOTE = Acetylation
  VARIANT 7: NOTE = D-Valine
  MOD_RES 12: NOTE = Lysine is bound to an albumn binding moiety
  VARIANT 32: NOTE = X = Thp
  MOD_RES 38: NOTE = Amidation

SEQ ID NO: 200 - protein, 38 aa, synthetic construct; identical to SEQ ID NO: 63
  SOURCE 1..38
  MOD_RES 1: NOTE = N-Methylated
  VARIANT 7: NOTE = D-Valine
  MOD_RES 12: NOTE = Lysine is bound to an labumin binding moiety
  VARIANT 23: NOTE = X = Aib
  VARIANT 32: NOTE = X = Aib
  MOD_RES 38: NOTE = Amidation

SEQ ID NO: 201 - protein, 37 aa, synthetic construct; identical to SEQ ID NO: 45
  SOURCE 1..37
  MOD_RES 1: NOTE = Acylation with Pentanoyl
  VARIANT 6: NOTE = D-Valine
  MOD_RES 11: NOTE = Lysine is bound to an albumin binding moiety
  VARIANT 31: NOTE = X = Aib
  MOD_RES 37: NOTE = Amidation

SEQ ID NO: 202 - protein, 37 aa, synthetic construct; identical to SEQ ID NO: 15
  SOURCE 1..37
  MOD_RES 1: NOTE = Acylation with Pentanoyl
  VARIANT 6: NOTE = D-Valine
  MOD_RES 11: NOTE = Lysine is bound to an albumin binding moiety
  VARIANT 22: NOTE = X = Aib
  VARIANT 31: NOTE = X = Aib

SEQ ID NO: 203 - protein, 38 aa, synthetic construct; identical to SEQ ID NO: 11
  SOURCE 1..38
  MOD_RES 1: NOTE = Acetylation
  VARIANT 7: NOTE = D-Valine
  MOD_RES 12: NOTE = Lysine is bound to an albumin binding moiety
  VARIANT 32: NOTE = X = Aib
  MOD_RES 38: NOTE = Amidation

SEQ ID NO: 204 - protein, 38 aa, synthetic construct; identical to SEQ ID NO: 11
  SOURCE 1..38
  MOD_RES 1: NOTE = Acetylation
  VARIANT 7: NOTE = D-Valine
  MOD_RES 12: NOTE = Lysine is bound to an albumin binding moiety
  VARIANT 32: NOTE = X = Aib
  MOD_RES 38: NOTE = Amidation

SEQ ID NO: 205 - protein, 38 aa, synthetic construct; identical to SEQ ID NO: 11
  SOURCE 1..38
  MOD_RES 1: NOTE = Acetylation
  VARIANT 7: NOTE = D-Valine
  MOD_RES 12: NOTE = Lysine is bound to an albumin binding moiety
  VARIANT 32: NOTE = X = Aib
  MOD_RES 38: NOTE = Amidation

SEQ ID NO: 206 - protein, 38 aa, synthetic construct; identical to SEQ ID NO: 11
  SOURCE 1..38
  MOD_RES 1: NOTE = Acetylation
  VARIANT 7: NOTE = D-Valine
  MOD_RES 12: NOTE = Lysine is bound to an albumin binding moiety
  VARIANT 32: NOTE = X = Aib
  MOD_RES 38: NOTE = Amidation

SEQ ID NO: 207 - protein, 38 aa, synthetic construct; identical to SEQ ID NO: 11
  SOURCE 1..38
  MOD_RES 1: NOTE = Acetylated
  VARIANT 7: NOTE = D-Valine
  MOD_RES 12: NOTE = Lysine is bound to an albumin binding moiety
  VARIANT 32: NOTE = X = 4-Pip
  MOD_RES 38: NOTE = Amidation

SEQ ID NO: 208 - protein, 38 aa, synthetic construct; identical to SEQ ID NO: 63
  SOURCE 1..38
  MOD_RES 1: NOTE = Acetylated
  VARIANT 7: NOTE = D-Valine
  MOD_RES 12: NOTE = Lysine is bound to an albumin binding moiety
  VARIANT 23: NOTE = X = Aib
  VARIANT 32: NOTE = X = 4-Pip
  MOD_RES 38: NOTE = Amidation

SEQ ID NO: 209 - protein, 38 aa, synthetic construct; identical to SEQ ID NO: 63
  SOURCE 1..38
  MOD_RES 1: NOTE = Acetylated
  VARIANT 7: NOTE = D-Valine
  MOD_RES 12: NOTE = Lysine is bound to an albumin binding moiety
  VARIANT 23: NOTE = X = Aib
  VARIANT 32: NOTE = X = Aib
  MOD_RES 38: NOTE = Amidation

SEQ ID NO: 210 - protein, 38 aa, synthetic construct; identical to SEQ ID NO: 11
  SOURCE 1..38
  MOD_RES 1: NOTE = Acetylated
  VARIANT 7: NOTE = D-Valine
  MOD_RES 12: NOTE = Lysine is bound to an albumin binding moiety
  VARIANT 32: NOTE = X = Thp
  MOD_RES 38: NOTE = Amidation

SEQ ID NO: 211 - protein, 38 aa, synthetic construct; identical to SEQ ID NO: 165
  SOURCE 1..38
  MOD_RES 1: NOTE = Acetylated
  VARIANT 7: NOTE = D-Valine
  MOD_RES 12: NOTE = Lysine is bound to an albumin binding moiety
  VARIANT 32: NOTE = X = Aib
  MOD_RES 38: NOTE = amidation

SEQ ID NO: 212 - protein, 38 aa, synthetic construct; identical to SEQ ID NO: 62
  SOURCE 1..38
  MOD_RES 1: NOTE = acetylated
  VARIANT 7: NOTE = D-Valine
  MOD_RES 12: NOTE = Lysine is bound to an albumin binding moiety
  VARIANT 32: NOTE = X = Aib
  MOD_RES 38: NOTE = Amidation

SEQ ID NO: 213 - protein, 38 aa, synthetic construct; identical to SEQ ID NO: 168
  SOURCE 1..38
  MOD_RES 1: NOTE = acetylated
  VARIANT 7: NOTE = D-Valine
  MOD_RES 12: NOTE = Lysine is bound to an albumin binding moiety
  VARIANT 32: NOTE = X = Aib
  MOD_RES 38: NOTE = Amidation

SEQ ID NO: 214 - protein, 38 aa, synthetic construct; identical to SEQ ID NO: 11
  SOURCE 1..38
  MOD_RES 1: NOTE = N-Methylation
  VARIANT 7: NOTE = D-Valine
  MOD_RES 12: NOTE = Lysine is bound to an albumin binding moiety
  VARIANT 32: NOTE = X = Aib
  MOD_RES 38: NOTE = Amidation

SEQ ID NO: 215 - protein, 38 aa, synthetic construct; identical to SEQ ID NO: 63
  SOURCE 1..38
  MOD_RES 1: NOTE = N-Methylated
  VARIANT 7: NOTE = D-Valine
  MOD_RES 12: NOTE = Lysine is bound to an albumin binding moiety
  VARIANT 23: NOTE = X = Aib
  VARIANT 32: NOTE = X = Aib
  MOD_RES 38: NOTE = Amidation

SEQ ID NO: 216 - protein, 38 aa, synthetic construct; identical to SEQ ID NO: 165
  SOURCE 1..38
  MOD_RES 1: NOTE = N-Methylated
  VARIANT 7: NOTE = D-Valine
  MOD_RES 12: NOTE = Lysine is bound to an albumin binding moiety
  VARIANT 32: NOTE = X = Aib
  MOD_RES 38: NOTE = Amidation

SEQ ID NO: 217 - protein, 38 aa, synthetic construct; identical to SEQ ID NO: 62
  SOURCE 1..38
  MOD_RES 1: NOTE = N-Methylated
  VARIANT 7: NOTE = D-Valine
  MOD_RES 12: NOTE = Lysine is bound to an albumin binding moiety
  VARIANT 32: NOTE = X = Aib
  MOD_RES 38: NOTE = Amidation

SEQ ID NO: 218 - protein, 38 aa, synthetic construct; identical to SEQ ID NO: 168
  SOURCE 1..38
  MOD_RES 1: NOTE = N-Methylated
  VARIANT 7: NOTE = D-Valine
  MOD_RES 12: NOTE = Lysine is bound to an albumin binding moiety
  VARIANT 32: NOTE = X = Aib
  MOD_RES 38: NOTE = Amidation

SEQ ID NO: 219 - protein, 37 aa, synthetic construct; identical to SEQ ID NO: 45
  SOURCE 1..37
  MOD_RES 1: NOTE = Acylated with Pentanoyl
  VARIANT 6: NOTE = D-Valine
  MOD_RES 11: NOTE = Lysine is bound to an albumin binding moiety
  VARIANT 31: NOTE = X = Aib
  MOD_RES 37: NOTE = Amidation

SEQ ID NO: 220 - protein, 37 aa, synthetic construct; identical to SEQ ID NO: 15
  SOURCE 1..37
  MOD_RES 1: NOTE = Acylated with Pentanoyl
  VARIANT 6: NOTE = D-Valine
  MOD_RES 11: NOTE = Lysine is bound to an albumin binding moiety
  VARIANT 22: NOTE = X = Aib
  VARIANT 31: NOTE = X = Aib
  MOD_RES 37: NOTE = Amidation

SEQ ID NO: 221 - protein, 37 aa, synthetic construct
  SOURCE 1..37
  MOD_RES 1: NOTE = Acylated with Pentanoyl
  VARIANT 6: NOTE = D-Valine
  MOD_RES 11: NOTE = Lysine is bound to an albumin binding moiety
  VARIANT 31: NOTE = X = Aib
  MOD_RES 37: NOTE = Amidation
VLSLDVPIKLKKILLEQEAQKKQREQAETNXQILAQV

SEQ ID NO: 222 - protein, 37 aa, synthetic construct
  SOURCE 1..37
  MOD_RES 1: NOTE = Acylated with Pentanoyl
  VARIANT 6: NOTE = D-Valine
  MOD_RES 11: NOTE = Lysine is bound to an albumin binding moiety
  VARIANT 31: NOTE = X = Aib
  MOD_RES 37: NOTE = Amidation
VLSLDVPIKLKKILLEQEKQKAQREQAETNXQILAQV

SEQ ID NO: 223 - protein, 37 aa, synthetic construct; identical to SEQ ID NO: 45
  SOURCE 1..37
  MOD_RES 1: NOTE = Acylation with Decanoyl
  VARIANT 6: NOTE = D-Valine
  MOD_RES 11: NOTE = Lysine is bound to an albumin binding moiety
  VARIANT 31: NOTE = X = Aib
  MOD_RES 37: NOTE = Amidation

SEQ ID NO: 224 - protein, 37 aa, synthetic construct; identical to SEQ ID NO: 45
  SOURCE 1..37
  MOD_RES 1: NOTE = Acylation with Dodecanoyl
  VARIANT 6: NOTE = D-Valine
  MOD_RES 11: NOTE = Lysine is bound to an albumin binding moiety
  VARIANT 31: NOTE = X = Aib
  MOD_RES 37: NOTE = Amidation

SEQ ID NO: 225 - protein, 37 aa, synthetic construct; identical to SEQ ID NO: 45
  SOURCE 1..37
  MOD_RES 1: NOTE = Acylation with Tetradecanoyl
  VARIANT 6: NOTE = D-Valine
  MOD_RES 11: NOTE = Lysine is bound to an albumin binding moiety
  VARIANT 31: NOTE = X = Aib
  MOD_RES 37: NOTE = Amidation

SEQ ID NO: 226 - protein, 38 aa, synthetic construct; identical to SEQ ID NO: 191
  SOURCE 1..38
  MOD_RES 1: NOTE = Acetylated
  VARIANT 7: NOTE = D-Valine
  MOD_RES 12: NOTE = Lysine is bound to an albumin binding moiety
  VARIANT 32: NOTE = X = Aib
  MOD_RES 38: NOTE = Amidation

SEQ ID NO: 227 - protein, 38 aa, synthetic construct; identical to SEQ ID NO: 191
  SOURCE 1..38
  MOD_RES 1: NOTE = Acetylated
  VARIANT 7: NOTE = D-Valine
  MOD_RES 12: NOTE = Lysine is bound to an albumin binding moiety
  VARIANT 32: NOTE = X = 4-Pip
  MOD_RES 38: NOTE = Amidation

SEQ ID NO: 228 - protein, 37 aa, synthetic construct; identical to SEQ ID NO: 195
  SOURCE 1..37
  MOD_RES 1: NOTE = Acylation with Pentanoyl
  VARIANT 6: NOTE = D-Valine
  MOD_RES 11: NOTE = Lysine is bound to an albumin binding moiety
  VARIANT 31: NOTE = X = Aib
  MOD_RES 37: NOTE = Amidation

SEQ ID NO: 229 - protein, 38 aa, synthetic construct; identical to SEQ ID NO: 191
  SOURCE 1..38
  MOD_RES 1: NOTE = N-Methylated
  VARIANT 7: NOTE = D-Valine
  MOD_RES 12: NOTE = Lysine is bound to an albumin binding moiety
  VARIANT 32: NOTE = X = Aib
  MOD_RES 38: NOTE = Amidation

SEQ ID NO: 230 - protein, 38 aa, synthetic construct; identical to SEQ ID NO: 11
  SOURCE 1..38
  MOD_RES 1: NOTE = Acetylated
  VARIANT 7: NOTE = D-Valine
  MOD_RES 12: NOTE = Lysine is bound to an albumin binding moiety
  VARIANT 32: NOTE = X = Aib
  MOD_RES 38: NOTE = Amidation

SEQ ID NO: 231 - protein, 38 aa, synthetic construct; identical to SEQ ID NO: 168
  SOURCE 1..38
  MOD_RES 1: NOTE = Acetylated
  VARIANT 7: NOTE = D-Valine
  MOD_RES 12: NOTE = Lysine is bound to an albumin binding moiety
  VARIANT 32: NOTE = X = Aib
  MOD_RES 38: NOTE = Amidation

SEQ ID NO: 232 - protein, 38 aa, synthetic construct; identical to SEQ ID NO: 62
  SOURCE 1..38
  MOD_RES 1: NOTE = Acetylated
  VARIANT 7: NOTE = D-Valine
  MOD_RES 12: NOTE = Lysine is bound to an albumin binding moiety
  VARIANT 32: NOTE = X = Aib
  MOD_RES 38: NOTE = Amidation

SEQ ID NO: 233 - protein, 38 aa, synthetic construct; identical to SEQ ID NO: 168
  SOURCE 1..38
  MOD_RES 1: NOTE = N-Methylated
  VARIANT 7: NOTE = D-Valine
  MOD_RES 12: NOTE = Lysine is bound to an albumin binding moiety
  VARIANT 32: NOTE = X = Aib
  MOD_RES 38: NOTE = Amidation

SEQ ID NO: 234 - protein, 38 aa, synthetic construct; identical to SEQ ID NO: 63
  SOURCE 1..38
  MOD_RES 1: NOTE = N-Methylated
  VARIANT 7: NOTE = D-Valine
  MOD_RES 12: NOTE = Lysine is bound to an albumin binding moiety
  VARIANT 32: NOTE = X = Aib
  MOD_RES 38: NOTE = Amidation
  VARIANT 23: NOTE = X = Aib

SEQ ID NO: 235 - protein, 37 aa, synthetic construct; identical to SEQ ID NO: 45
  SOURCE 1..37
  MOD_RES 1: NOTE = Acylation with Pentanoyl
  VARIANT 6: NOTE = D-Valine
  MOD_RES 11: NOTE = Lysine is bound to an albumin binding moiety
  VARIANT 31: NOTE = X = Aib
  MOD_RES 37: NOTE = Amidation

SEQ ID NO: 236 - protein, 38 aa, synthetic construct; identical to SEQ ID NO: 168
  SOURCE 1..38
  MOD_RES 1: NOTE = Acetylated
  VARIANT 7: NOTE = D-Valine
  MOD_RES 12: NOTE = Lysine is bound to an albumin binding moiety
  VARIANT 32: NOTE = X = Aib
  MOD_RES 38: NOTE = Amidation

SEQ ID NO: 237 - protein, 38 aa, synthetic construct; identical to SEQ ID NO: 168
  SOURCE 1..38
  MOD_RES 1: NOTE = N-Methylated
  VARIANT 7: NOTE = D-Valine
  MOD_RES 12: NOTE = Lysine is bound to an albumin binding moiety
  VARIANT 32: NOTE = X = Aib
  MOD_RES 38: NOTE = Amidation

SEQ ID NO: 238 - protein, 38 aa, synthetic construct; identical to SEQ ID NO: 11
  SOURCE 1..38
  MOD_RES 1: NOTE = Acetylated
  VARIANT 7: NOTE = D-Valine
  MOD_RES 12: NOTE = Lysine is bound to an albumin binding moiety
  VARIANT 32: NOTE = X = Aib
  MOD_RES 38: NOTE = Amidation

SEQ ID NO: 239 - protein, 38 aa, synthetic construct; identical to SEQ ID NO: 63
  SOURCE 1..38
  MOD_RES 1: NOTE = N-Methylated
  VARIANT 7: NOTE = D-Valine
  MOD_RES 12: NOTE = Lysine is bound to an albumin binding moiety
  VARIANT 23: NOTE = X = Aib
  VARIANT 32: NOTE = X = Aib
  MOD_RES 38: NOTE = Amidation

SEQ ID NO: 240 - protein, 38 aa, synthetic construct; identical to SEQ ID NO: 62
  SOURCE 1..38
  MOD_RES 1: NOTE = Acetylated
  VARIANT 7: NOTE = D-Valine
  MOD_RES 12: NOTE = Lysine is bound to an albumin binding moiety
  VARIANT 32: NOTE = X = Aib
  MOD_RES 38: NOTE = Amidation

SEQ ID NO: 241 - protein, 38 aa, synthetic construct; identical to SEQ ID NO: 168
  SOURCE 1..38
  MOD_RES 1: NOTE = Acetylated
  VARIANT 7: NOTE = D-Valine
  MOD_RES 12: NOTE = Lysine is bound to an albumin binding moiety
  VARIANT 32: NOTE = X = Aib
  MOD_RES 38: NOTE = Amidation

SEQ ID NO: 242 - protein, 38 aa, synthetic construct; identical to SEQ ID NO: 168
  SOURCE 1..38
  MOD_RES 1: NOTE = N-Methylated
  VARIANT 7: NOTE = D-Valine
  MOD_RES 12: NOTE = Lysine is bound to an albumin binding moiety
  VARIANT 32: NOTE = X = Aib
  MOD_RES 38: NOTE = Amidation

SEQ ID NO: 243 - protein, 38 aa, synthetic construct; identical to SEQ ID NO: 11
  SOURCE 1..38
  MOD_RES 1: NOTE = Acetylated
  VARIANT 7: NOTE = D-Valine
  MOD_RES 12: NOTE = Lysine is bound to an albumin binding moiety
  VARIANT 32: NOTE = X = Aib
  MOD_RES 38: NOTE = Amidation

SEQ ID NO: 244 - protein, 38 aa, synthetic construct; identical to SEQ ID NO: 62
  SOURCE 1..38
  MOD_RES 1: NOTE = Acetylated
  VARIANT 7: NOTE = D-Valine
  MOD_RES 12: NOTE = Lysine is bound to an albumin binding moiety
  VARIANT 32: NOTE = X = Aib
  MOD_RES 38: NOTE = Amidation